European Patent Specification EP 3 615 566 B1, published December 20, 2023. Title: MULTISPECIFIC MOLECULES COMPRISING A NON-IMMUNOGLOBULIN HETERODIMERIZATION DOMAIN AND USES THEREOF. Applicant: ELSTAR THERAPEUTICS, INC. The sequence listing filed with the application follows.

SEQUENCE LISTING (171 sequences)

SEQ ID NO: 1 - protein, 93 aa, Homo sapiens
PDIQNPDPAVYQLRDSKSSDKSVCLFTDFDSQTNVSQSKDSDVYITDKCVLDMRSMDFKSNSAVAWSNKSDFACANAFNNSIIPEDTFFPSPE

SEQ ID NO: 2 - protein, 130 aa, Homo sapiens
EDLNKVFPPEVALFEPSEAEISHTQKATLVCLATGFYPDHVELSWWVNGKEVHSGVCTDPQPLKEQPALNDSRYALSSRLRVSATFWQDPRNHFRCQVQFYGLSEADEWTQARAKPVTQIVSAEAWGRAD

SEQ ID NO: 3-4 - skipped (2 entries)

SEQ ID NO: 5 - protein, 114 aa, Homo sapiens
NWVNVISDLKKIEDLIQSMHIDATLYTESDVHPSCKVTAMKCFLLELQVISLESGDASIHDTVENLIILANNSLSSNGNVTESGCKECEELEEKNIKEFLQSFVHIVQMFINTS

SEQ ID NO: 6 - protein, 77 aa, Artificial Sequence
  source: /note="Description of Artificial Sequence: Synthetic polypeptide"
MAPRRARGCRTLGLPALLLLLLLRPPATRGITCPPPMSVEHADIWVKSYSLYSRERYICNSGFKRKAGTSSLTECVL

SEQ ID NO: 7 - protein, 20 aa, Artificial Sequence
  source: /note="Description of Artificial Sequence: Synthetic peptide"
SGGSGGGGSGGGSGGGGSLQ

SEQ ID NO: 8 - protein, 133 aa, Homo sapiens [sequence omitted]

SEQ ID NO: 9 - protein, 157 aa, Homo sapiens
YFGKLESKLSVIRNLNDQVLFIDQGNRPLFEDMTDSDCRDNAPRTIFIISMYKDSQPRGMAVTISVKCEKISTLSCENKIISFKEMNPPDNIKDTKSDIIFFQRSVPGHDNKMQFESSSYEGYFLACEKERDLFKLILKKEDELGDRSIMFTVQNED

SEQ ID NO: 10 - protein, 133 aa, Homo sapiens [sequence omitted]

SEQ ID NO: 11 - protein, 138 aa, Homo sapiens
QDPYVKEAENLKKYFNAGHSDVADNGTLFLGILKNWKEESDRKIMQSQIVSFYFKLFKNFKDDQSIQKSVETIKEDMNVKFFNSNKKKRDDFEKLTNYSVTDLNVQRKAIHELIQVMAELSPAAKTGKRKRSQMLFRG

SEQ ID NO: 12 - protein, 454 aa, Artificial Sequence
  source: /note="Description of Artificial Sequence: Synthetic polypeptide"
METDTLLLWVLLLWVPGSTGQVQLVESGGGVVQPGRSLRLSCAASGFTFSSYTMHWVRQAPGKGLEWVTFISYDGNNKYYADSVKGRFTISRDNSKNTLYLQMNSLRAEDTAIYYCARTGWLGPFDYWGQGTLVTVSSASTKGPSVFPLAPSSKSTSGGTAALGCLVKDYFPEPVTVSWNSGALTSGVHTFPAVLQSSGLYSLSSVVTVPSSSLGTQTYICNVNHKPSNTKVDKRVEPKSCDKTHTCPPCPAPELLGGPSVFLFPPKPKDTLMISRTPEVTCVVVDVSHEDPEVKFNWYVDGVEVHNAKTKPREEQYNSTYRVVSVLTVLHQDWLNGKEYKCKVSNKALPAPIEKTISKAKPDIQNPDPAVYQLRDSKSSDKSVCLFTDFDSQTNVSQSKDSDVYITDKCVLDMRSMDFKSNSAVAWSNKSDFACANAFNNSIIPEDTFFPSPE

SEQ ID NO: 13 - protein, 488 aa, Artificial Sequence
  source: /note="Description of Artificial Sequence: Synthetic polypeptide"
METDTLLLWVLLLWVPGSTGQVQLVESGGGVVQPGRSLRLSCAASGFTFSSYGMHWVRQAPGKGLEWVAFIRYDGSNKYYADSVKGRFTISRDNSKNTLYLQMNSLRAEDTAVYYCKTHGSHDNWGQGTMVTVSSASTKGPSVFPLAPSSKSTSGGTAALGCLVKDYFPEPVTVSWNSGALTSGVHTFPAVLQSSGLYSLSSVVTVPSSSLGTQTYICNVNHKPSNTKVDKRVEPKSCDKTHTCPPCPAPELLGGPSVFLFPPKPKDTLMISRTPEVTCVVVDVSHEDPEVKFNWYVDGVEVHNAKTKPREEQYNSTYRVVSVLTVLHQDWLNGKEYKCKVSNKALPAPIEKTISKAKEDLNKVFPPEVALFEPSEAEISHTQKATLVCLATGFYPDHVELSWWVNGKEVHSGVCTDPQPLKEQPALNDSRYALSSRLRVSATFWQDPRNHFRCQVQFYGLSEADEWTQARAKPVTQIVSAEAWGRAD

SEQ ID NO: 14 - protein, 235 aa, Artificial Sequence
  source: /note="Description of Artificial Sequence: Synthetic polypeptide"
METDTLLLWVLLLWVPGSTGEIVLTQSPGTLSLSPGERATLSCRASQSVGSSYLAWYQQKPGQAPRLLIYGAFSRATGIPDRFSGSGSGTDFTLTISRLEPEDFAVYYCQQYGSSPWTFGQGTKVEIKRTVAAPSVFIFPPSDEQLKSGTASVVCLLNNFYPREAKVQWKVDNALQSGNSQESVTEQDSKDSTYSLSSTLTLSKADYEKHKVYACEVTHQGLSSPVTKSFNRGEC

SEQ ID NO: 15 - protein, 237 aa, Artificial Sequence
  source: /note="Description of Artificial Sequence: Synthetic polypeptide"
METDTLLLWVLLLWVPGSTGQSVLTQPPSVSGAPGQRVTISCSGSRSNIGSNTVKWYQQLPGTAPKLLIYYNDQRPSGVPDRFSGSKSGTSASLAITGLQAEDEADYYCQSYDRYTHPALLFGTGTKVTVLGQPKANPTVTLFPPSSEELQANKATLVCLISDFYPGAVTVAWKADGSPVKAGVETTKPSKQSNNKYAASSYLSLTPEQWKSHRSYSCQVTHEGSTVEKTVAPTECS

SEQ ID NO: 16 - DNA, 354 bp, Artificial Sequence
  source: /note="Description of Artificial Sequence: Synthetic polynucleotide"
caggtgcagctggtggaatctggtggcggagttgtgcagcctggcagatccctgagactgtcttgtgccgcctccggcttcaccttctccagctacaccatgcactgggtccgacaggcccctggcaaaggattggagtgggtcaccttcatctcttacgacggcaacaacaagtactacgccgactccgtgaagggcagattcaccatctctcgggacaactccaagaacaccctgtacctgcagatgaactccctgagagccgaggacaccgccatctactactgtgctagaaccggctggctgggcccctttgattattggggacagggcaccctggtcaccgtgtcctct

SEQ ID NO: 17 - DNA, 324 bp, Artificial Sequence
  source: /note="Description of Artificial Sequence: Synthetic polynucleotide"
gagatcgtgctgacccagtctcctggcacactgtcactgtctccaggcgagagagctaccctgtcctgtagagcctctcagtccgtgggctcctcttacctggcttggtatcagcagaagcccggccaggctcctagactgttgatctacggcgccttctccagagccacaggcatccctgatagattctccggctctggctctggcaccgacttcaccctgaccatctccagactggaacccgaggacttcgccgtgtactactgtcagcagtacggctcctctccttggacctttggccagggcaccaaggtggaaatcaag

SEQ ID NO: 18 - DNA, 345 bp, Artificial Sequence
  source: /note="Description of Artificial Sequence: Synthetic polynucleotide"
caggtgcagctggtggaatctggtggcggagttgtgcagcctggcagatccctgagactgtcttgtgccgcctccggcttcaccttctcctcttacggaatgcactgggtccgacaggcccctggcaaaggattggagtgggtcgccttcatcagatacgacggctccaacaagtactacgccgactccgtgaagggcagattcaccatctctcgggacaactccaagaacaccctgtacctgcagatgaactccctgagagccgaggacaccgccgtgtactactgcaagacccacggctctcacgacaattggggccagggcacaatggtcaccgtgtcctct

SEQ ID NO: 19 - DNA, 333 bp, Artificial Sequence
  source: /note="Description of Artificial Sequence: Synthetic polynucleotide"
cagtccgtgttgacccagcctccttctgtttctggcgctcctggccagagagtgaccatctcttgctccggctctcggtccaacatcggctccaataccgtgaagtggtatcagcagctgcccggcacagctcccaaactgctgatctactacaacgaccagcggccttctggcgtgcccgatagattctctggctccaagtctggcacctctgccagcctggctattaccggactgcaggctgaggacgaggccgactactactgccagtcttacgaccggtacacccatcctgctctgctgtttggcaccggcaccaaagtgacagtgctg

SEQ ID NO: 20 - DNA, 321 bp, Artificial Sequence
  source: /note="Description of Artificial Sequence: Synthetic polynucleotide"
cggacagtggccgctccttccgtgttcatcttcccaccttccgacgagcagctgaagtccggcacagcttctgtcgtgtgcctgctgaacaacttctaccctcgggaagccaaggtgcagtggaaggtggacaatgccctgcagtccggcaactcccaagagtctgtgaccgagcaggactccaaggacagcacctacagcctgtcctccacactgaccctgtccaaggccgactacgagaagcacaaggtgtacgcctgcgaagtgacccatcagggcctgtctagccctgtgaccaagtctttcaaccggggcgagtgc

SEQ ID NO: 21 - DNA, 318 bp, Artificial Sequence
  source: /note="Description of Artificial Sequence: Synthetic polynucleotide"
ggccagcctaaggccaatcctaccgtgacactgttccctccatcctccgaagaactgcaggccaacaaggctaccctcgtgtgcctgatctccgacttttaccctggcgctgtgaccgtggcctggaaggctgatggatctcctgtgaaggctggcgtggaaaccaccaagccttccaagcagtccaacaacaaatacgccgcctcctcctacctgtctctgacccctgaacagtggaagtcccaccggtcctacagctgccaagtgacccatgagggctccaccgtggaaaagaccgtggctcctaccgagtgctcc

SEQ ID NO: 22 - DNA, 309 bp, Artificial Sequence
  source: /note="Description of Artificial Sequence: Synthetic polynucleotide"
gcttccaccaagggaccctctgtgttccctctggctccttccagcaagtctacctctggcggaacagctgctctgggctgcctggtcaaggactactttcctgagcctgtgaccgtgtcttggaactctggcgctctgacatccggcgtgcacacctttccagctgtgctgcaatcctccggcctgtactctctgtcctccgtcgtgaccgtgccttctagctctctgggcacccagacctacatctgcaatgtgaaccacaagccttccaacaccaaggtggacaagagagtggaacccaagtcctgc

SEQ ID NO: 23 - DNA, 360 bp, Artificial Sequence
  source: /note="Description of Artificial Sequence: Synthetic polynucleotide"
gataagacccacacctgtccaccatgtcctgctccagaactgctcggcggaccttccgtgttcctgtttcctccaaagcctaaggacaccctgatgatctctcggacccctgaagtgacctgcgtggtggtggatgtgtctcacgaggatcccgaagtgaagttcaattggtacgtggacggcgtggaagtgcacaacgccaagaccaagcctagagaggaacagtacaactccacctacagagtggtgtccgtgctgaccgtgctgcaccaggattggctgaacggcaaagagtacaagtgcaaggtgtccaacaaggccctgcctgctcctatcgaaaagaccatctccaaggccaaa

SEQ ID NO: 24 - DNA, 279 bp, Artificial Sequence
  source: /note="Description of Artificial Sequence: Synthetic polynucleotide"
cctgacattcagaaccccgatcctgccgtgtaccagctgagagactccaagtcctccgataagtctgtgtgcctgttcaccgacttcgactcccagaccaacgtgtcccagtccaaggactccgacgtgtacatcaccgataagtgcgtgctggacatgcggagcatggacttcaagtctaactccgccgtggcctggtctaacaagtccgatttcgcctgcgccaacgccttcaacaacagcattatccccgaggacacattcttcccatcacctgag

SEQ ID NO: 25 - DNA, 390 bp, Artificial Sequence
  source: /note="Description of Artificial Sequence: Synthetic polynucleotide"
gaggacctgaacaaggttttcccacctgaggtggccctgttcgagccttctgaggctgagatctctcacacccagaaagctaccctcgtgtgtctggccaccggcttctaccctgatcacgtggaactgtcttggtgggtcaacggaaaagaggtgcactccggcgtctgcaccgatcctcagcctctgaaagaacagcccgctctgaacgactccagatacgccctgtcctctcggctgagagtgtctgccaccttctggcaggaccctcggaaccactttagatgccaggtgcagttctacggcctgtccgaggctgatgagtggacccaggctagagccaagccagtgacacagatcgtgtctgccgaagcctggggcagagccgat

SEQ ID NO: 26 - DNA, 3 bp, Artificial Sequence
  source: /note="Description of Artificial Sequence: Synthetic oligonucleotide"
ggt

SEQ ID NO: 27 - DNA, 6 bp, Artificial Sequence
  source: /note="Description of Artificial Sequence: Synthetic oligonucleotide"
ggtggc

SEQ ID NO: 28 - DNA, 9 bp, Artificial Sequence
  source: /note="Description of Artificial Sequence: Synthetic oligonucleotide"
ggtggcgga

SEQ ID NO: 29 - DNA, 12 bp, Artificial Sequence
  source: /note="Description of Artificial Sequence: Synthetic oligonucleotide"
ggtggcggagga

SEQ ID NO: 30 - DNA, 15 bp, Artificial Sequence
  source: /note="Description of Artificial Sequence: Synthetic oligonucleotide"
ggtggcggaggaagc

SEQ ID NO: 31 - DNA, 18 bp, Artificial Sequence
  source: /note="Description of Artificial Sequence: Synthetic oligonucleotide"
ggtggcggaggaagcggt

SEQ ID NO: 32 - DNA, 21 bp, Artificial Sequence
  source: /note="Description of Artificial Sequence: Synthetic oligonucleotide"
ggtggcggaggaagcggtggc

SEQ ID NO: 33 - DNA, 24 bp, Artificial Sequence
  source: /note="Description of Artificial Sequence: Synthetic oligonucleotide"
ggtggcggaggaagcggtggcggc

SEQ ID NO: 34 - DNA, 27 bp, Artificial Sequence
  source: /note="Description of Artificial Sequence: Synthetic oligonucleotide"
ggtggcggaggaagcggtggcggcgga

SEQ ID NO: 35 - DNA, 30 bp, Artificial Sequence
  source: /note="Description of Artificial Sequence: Synthetic oligonucleotide"
ggtggcggaggaagcggtggcggcggatct

SEQ ID NO: 36 - DNA, 360 bp, Artificial Sequence
  source: /note="Description of Artificial Sequence: Synthetic polynucleotide"
accatcaagccttgtcctccatgcaagtgccccgctcctaatctgctcggaggcccttccgtgttcatcttcccacctaagatcaaggacgtgctgatgatctccctgtctcctatcgtgacctgcgtggtggtggacgtgtccgaggatgatcctgacgtgcagatcagttggttcgtgaacaacgtggaagtgcacaccgctcagacccagacacacagagaggactacaacagcaccctgagagtggtgtctgccctgcctatccagcaccaggattggatgtccggcaaagaattcaagtgcaaagtgaacaacaaggacctgcctgctccaatcgagcggaccatctccaagcct

SEQ ID NO: 37 - DNA, 348 bp, Artificial Sequence
  source: /note="Description of Artificial Sequence: Synthetic polynucleotide"
aagcctaacatccagaatcctgagcctgccgtgtaccagctgaaggaccctagatctcaggactctaccctgtgcctgttcaccgacttcgactcccagatcaacgtgcccaagaccatggaatccggcaccttcatcaccgataagtgcgtgctggacatgaaggccatggactccaagtccaacggcgctatcgcctggtccaaccagaccagcttcacatgccaggacatcttcaaagagacaaacgccacctatccttccagcgacgtgccctgtgatgctaccctgaccgagaagtccttcgagacagacatgaacctgaacttccagaacctgtcctgatga

SEQ ID NO: 38 - DNA, 390 bp, Artificial Sequence
  source: /note="Description of Artificial Sequence: Synthetic polynucleotide"
gtggtggaagatctgcggaacgtgacccctcctaaggtgtccctgttcgagccttccaaggccgagatcgccaacaagcagaaagctaccctcgtgtgcctggccagaggcttctttcctgaccacgtggaactgtcttggtgggtcaacggcaaagaggtgcactccggcgtctgtaccgatcctcaggcctacaaagagtccaactactcctacagcctgtcctctcggctgagagtgtctgccaccttctggcacaaccctcggaaccacttcagatgccaggtgcagtttcacggcctgtccgaagaggacaagtggcctgagggatcccctaagcctgtgacacagaacatctctgccgaggcctggggtagagctgatggtggc

SEQ ID NO: 39 - DNA, 372 bp, Artificial Sequence
  source: /note="Description of Artificial Sequence: Synthetic polynucleotide"
ctggaacagctgctgatggacctgcaagagctgctgtcccggatggaaaactaccggaacctgaagctgccccggatgctgaccgctaagttcgctctgcctaagcaggccaccgagctgaaggatctgcagtgcctggaagatgagctgggccctctgagacacgtgctggatctgacccagtccaagtcctttcagctcgaggacgccgagaacttcatctccaacatcagagtgaccgtggtcaagctgaagggctccgacaacaccttcgagtgccagttcgacgatgagtccgctacagtggtggacttcctgcggagatggatcgccttctgccagtccatcatctccacctctccacagtgatga

SEQ ID NO: 40 - DNA, 45 bp, Artificial Sequence
  source: /note="Description of Artificial Sequence: Synthetic oligonucleotide"
ggaggatctggcggaggtggaagcggcggaggcggatcttctcat

SEQ ID NO: 41 - DNA, 321 bp, Artificial Sequence
  source: /note="Description of Artificial Sequence: Synthetic polynucleotide"
ggccagcctagggaaccccaggtttacaccctgcctccatgccgggaagagatgaccaagaaccaggtgtccctgtggtgcctggttaagggcttctacccctccgatatcgccgtggaatgggagtctaatggccagcctgagaacaactacaagacaacccctcctgtgctggactccgacggctcattcttcctgtactccaagctgacagtggacaagtccagatggcagcagggcaacgtgttctcctgctccgtgatgcacgaggccctgcacaatcactacacccagaagtccctgtctctgagccccggcaag

SEQ ID NO: 42 - DNA, 320 bp, Artificial Sequence
  source: /note="Description of Artificial Sequence: Synthetic polynucleotide"
gccagcctcgggaacctcaagtctgtaccctgcctcctagccgggaagagatgaccaagaaccaggtgtccctgtcctgcgctgtgaagggcttctacccttccgatatcgccgtggaatgggagagcaatggccagcctgagaacaactacaagaccacacctcctgtgctggactccgacggctcattcttcctggtgtccaagctgacagtggacaagtccagatggcagcagggcaacgtgttctcctgctccgtgatgcacgaggccctgcacaatcactacacccagaagtccctgtctctgagccccggcaag

SEQ ID NO: 43 - DNA, 1302 bp, Artificial Sequence
  source: /note="Description of Artificial Sequence: Synthetic polynucleotide"
caggtgcagctggtggaatctggtggcggagttgtgcagcctggcagatccctgagactgtcttgtgccgcctccggcttcaccttctccagctacaccatgcactgggtccgacaggcccctggcaaaggattggagtgggtcaccttcatctcttacgacggcaacaacaagtactacgccgactccgtgaagggcagattcaccatctctcgggacaactccaagaacaccctgtacctgcagatgaactccctgagagccgaggacaccgccatctactactgtgctagaaccggctggctgggcccctttgattattggggacagggcaccctggtcaccgtgtcctctgcttccaccaagggaccctctgtgttccctctggctccttccagcaagtctacctctggcggaacagctgctctgggctgcctggtcaaggactactttcctgagcctgtgaccgtgtcttggaactctggcgctctgacatccggcgtgcacacctttccagctgtgctgcaatcctccggcctgtactctctgtcctccgtcgtgaccgtgccttctagctctctgggcacccagacctacatctgcaatgtgaaccacaagccttccaacaccaaggtggacaagagagtggaacccaagtcctgcgataagacccacacctgtccaccatgtcctgctccagaactgctcggcggaccttccgtgttcctgtttcctccaaagcctaaggacaccctgatgatctctcggacccctgaagtgacctgcgtggtggtggatgtgtctcacgaggatcccgaagtgaagttcaattggtacgtggacggcgtggaagtgcacaacgccaagaccaagcctagagaggaacagtacaactccacctacagagtggtgtccgtgctgaccgtgctgcaccaggattggctgaacggcaaagagtacaagtgcaaggtgtccaacaaggccctgcctgctcctatcgaaaagaccatctccaaggccaaacctgacattcagaaccccgatcctgccgtgtaccagctgagagactccaagtcctccgataagtctgtgtgcctgttcaccgacttcgactcccagaccaacgtgtcccagtccaaggactccgacgtgtacatcaccgataagtgcgtgctggacatgcggagcatggacttcaagtctaactccgccgtggcctggtctaacaagtccgatttcgcctgcgccaacgccttcaacaacagcattatccccgaggacacattcttcccatcacctgag

SEQ ID NO: 44 - DNA, 1305 bp, Artificial Sequence
  source: /note="Description of Artificial Sequence: Synthetic polynucleotide"
caggtgcagctggtggaatctggtggcggagttgtgcagcctggcagatccctgagactgtcttgtgccgcctccggcttcaccttctccagctacaccatgcactgggtccgacaggcccctggcaaaggattggagtgggtcaccttcatctcttacgacggcaacaacaagtactacgccgactccgtgaagggcagattcaccatctctcgggacaactccaagaacaccctgtacctgcagatgaactccctgagagccgaggacaccgccatctactactgtgctagaaccggctggctgggcccctttgattattggggacagggcaccctggtcaccgtgtcctctgcttccaccaagggaccctctgtgttccctctggctccttccagcaagtctacctctggcggaacagctgctctgggctgcctggtcaaggactactttcctgagcctgtgaccgtgtcttggaactctggcgctctgacatccggcgtgcacacctttccagctgtgctgcaatcctccggcctgtactctctgtcctccgtcgtgaccgtgccttctagctctctgggcacccagacctacatctgcaatgtgaaccacaagccttccaacaccaaggtggacaagagagtggaacccaagtcctgcgataagacccacacctgtccaccatgtcctgctccagaactgctcggcggaccttccgtgttcctgtttcctccaaagcctaaggacaccctgatgatctctcggacccctgaagtgacctgcgtggtggtggatgtgtctcacgaggatcccgaagtgaagttcaattggtacgtggacggcgtggaagtgcacaacgccaagaccaagcctagagaggaacagtacaactccacctacagagtggtgtccgtgctgaccgtgctgcaccaggattggctgaacggcaaagagtacaagtgcaaggtgtccaacaaggccctgcctgctcctatcgaaaagaccatctccaaggccaaaggtcctgacattcagaaccccgatcctgccgtgtaccagctgagagactccaagtcctccgataagtctgtgtgcctgttcaccgacttcgactcccagaccaacgtgtcccagtccaaggactccgacgtgtacatcaccgataagtgcgtgctggacatgcggagcatggacttcaagtctaactccgccgtggcctggtctaacaagtccgatttcgcctgcgccaacgccttcaacaacagcattatccccgaggacacattcttcccatcacctgag

SEQ ID NO: 45 - DNA, 1308 bp, Artificial Sequence
  source: /note="Description of Artificial Sequence: Synthetic polynucleotide"
caggtgcagctggtggaatctggtggcggagttgtgcagcctggcagatccctgagactgtcttgtgccgcctccggcttcaccttctccagctacaccatgcactgggtccgacaggcccctggcaaaggattggagtgggtcaccttcatctcttacgacggcaacaacaagtactacgccgactccgtgaagggcagattcaccatctctcgggacaactccaagaacaccctgtacctgcagatgaactccctgagagccgaggacaccgccatctactactgtgctagaaccggctggctgggcccctttgattattggggacagggcaccctggtcaccgtgtcctctgcttccaccaagggaccctctgtgttccctctggctccttccagcaagtctacctctggcggaacagctgctctgggctgcctggtcaaggactactttcctgagcctgtgaccgtgtcttggaactctggcgctctgacatccggcgtgcacacctttccagctgtgctgcaatcctccggcctgtactctctgtcctccgtcgtgaccgtgccttctagctctctgggcacccagacctacatctgcaatgtgaaccacaagccttccaacaccaaggtggacaagagagtggaacccaagtcctgcgataagacccacacctgtccaccatgtcctgctccagaactgctcggcggaccttccgtgttcctgtttcctccaaagcctaaggacaccctgatgatctctcggacccctgaagtgacctgcgtggtggtggatgtgtctcacgaggatcccgaagtgaagttcaattggtacgtggacggcgtggaagtgcacaacgccaagaccaagcctagagaggaacagtacaactccacctacagagtggtgtccgtgctgaccgtgctgcaccaggattggctgaacggcaaagagtacaagtgcaaggtgtccaacaaggccctgcctgctcctatcgaaaagaccatctccaaggccaaaggtggccctgacattcagaaccccgatcctgccgtgtaccagctgagagactccaagtcctccgataagtctgtgtgcctgttcaccgacttcgactcccagaccaacgtgtcccagtccaaggactccgacgtgtacatcaccgataagtgcgtgctggacatgcggagcatggacttcaagtctaactccgccgtggcctggtctaacaagtccgatttcgcctgcgccaacgccttcaacaacagcattatccccgaggacacattcttcccatcacctgag

SEQ ID NO: 46 - DNA, 1311 bp, Artificial Sequence
  source: /note="Description of Artificial Sequence: Synthetic polynucleotide"
caggtgcagctggtggaatctggtggcggagttgtgcagcctggcagatccctgagactgtcttgtgccgcctccggcttcaccttctccagctacaccatgcactgggtccgacaggcccctggcaaaggattggagtgggtcaccttcatctcttacgacggcaacaacaagtactacgccgactccgtgaagggcagattcaccatctctcgggacaactccaagaacaccctgtacctgcagatgaactccctgagagccgaggacaccgccatctactactgtgctagaaccggctggctgggcccctttgattattggggacagggcaccctggtcaccgtgtcctctgcttccaccaagggaccctctgtgttccctctggctccttccagcaagtctacctctggcggaacagctgctctgggctgcctggtcaaggactactttcctgagcctgtgaccgtgtcttggaactctggcgctctgacatccggcgtgcacacctttccagctgtgctgcaatcctccggcctgtactctctgtcctccgtcgtgaccgtgccttctagctctctgggcacccagacctacatctgcaatgtgaaccacaagccttccaacaccaaggtggacaagagagtggaacccaagtcctgcgataagacccacacctgtccaccatgtcctgctccagaactgctcggcggaccttccgtgttcctgtttcctccaaagcctaaggacaccctgatgatctctcggacccctgaagtgacctgcgtggtggtggatgtgtctcacgaggatcccgaagtgaagttcaattggtacgtggacggcgtggaagtgcacaacgccaagaccaagcctagagaggaacagtacaactccacctacagagtggtgtccgtgctgaccgtgctgcaccaggattggctgaacggcaaagagtacaagtgcaaggtgtccaacaaggccctgcctgctcctatcgaaaagaccatctccaaggccaaaggtggcggacctgacattcagaaccccgatcctgccgtgtaccagctgagagactccaagtcctccgataagtctgtgtgcctgttcaccgacttcgactcccagaccaacgtgtcccagtccaaggactccgacgtgtacatcaccgataagtgcgtgctggacatgcggagcatggacttcaagtctaactccgccgtggcctggtctaacaagtccgatttcgcctgcgccaacgccttcaacaacagcattatccccgaggacacattcttcccatcacctgag

SEQ ID NO: 47 - DNA, 1314 bp, Artificial Sequence
  source: /note="Description of Artificial Sequence: Synthetic polynucleotide"
caggtgcagctggtggaatctggtggcggagttgtgcagcctggcagatccctgagactgtcttgtgccgcctccggcttcaccttctccagctacaccatgcactgggtccgacaggcccctggcaaaggattggagtgggtcaccttcatctcttacgacggcaacaacaagtactacgccgactccgtgaagggcagattcaccatctctcgggacaactccaagaacaccctgtacctgcagatgaactccctgagagccgaggacaccgccatctactactgtgctagaaccggctggctgggcccctttgattattggggacagggcaccctggtcaccgtgtcctctgcttccaccaagggaccctctgtgttccctctggctccttccagcaagtctacctctggcggaacagctgctctgggctgcctggtcaaggactactttcctgagcctgtgaccgtgtcttggaactctggcgctctgacatccggcgtgcacacctttccagctgtgctgcaatcctccggcctgtactctctgtcctccgtcgtgaccgtgccttctagctctctgggcacccagacctacatctgcaatgtgaaccacaagccttccaacaccaaggtggacaagagagtggaacccaagtcctgcgataagacccacacctgtccaccatgtcctgctccagaactgctcggcggaccttccgtgttcctgtttcctccaaagcctaaggacaccctgatgatctctcggacccctgaagtgacctgcgtggtggtggatgtgtctcacgaggatcccgaagtgaagttcaattggtacgtggacggcgtggaagtgcacaacgccaagaccaagcctagagaggaacagtacaactccacctacagagtggtgtccgtgctgaccgtgctgcaccaggattggctgaacggcaaagagtacaagtgcaaggtgtccaacaaggccctgcctgctcctatcgaaaagaccatctccaaggccaaaggtggcggaggacctgacattcagaaccccgatcctgccgtgtaccagctgagagactccaagtcctccgataagtctgtgtgcctgttcaccgacttcgactcccagaccaacgtgtcccagtccaaggactccgacgtgtacatcaccgataagtgcgtgctggacatgcggagcatggacttcaagtctaactccgccgtggcctggtctaacaagtccgatttcgcctgcgccaacgccttcaacaacagcattatccccgaggacacattcttcccatcacctgag

SEQ ID NO: 48 - DNA, 1317 bp, Artificial Sequence
  source: /note="Description of Artificial Sequence: Synthetic polynucleotide"
caggtgcagctggtggaatctggtggcggagttgtgcagcctggcagatccctgagactgtcttgtgccgcctccggcttcaccttctccagctacaccatgcactgggtccgacaggcccctggcaaaggattggagtgggtcaccttcatctcttacgacggcaacaacaagtactacgccgactccgtgaagggcagattcaccatctctcgggacaactccaagaacaccctgtacctgcagatgaactccctgagagccgaggacaccgccatctactactgtgctagaaccggctggctgggcccctttgattattggggacagggcaccctggtcaccgtgtcctctgcttccaccaagggaccctctgtgttccctctggctccttccagcaagtctacctctggcggaacagctgctctgggctgcctggtcaaggactactttcctgagcctgtgaccgtgtcttggaactctggcgctctgacatccggcgtgcacacctttccagctgtgctgcaatcctccggcctgtactctctgtcctccgtcgtgaccgtgccttctagctctctgggcacccagacctacatctgcaatgtgaaccacaagccttccaacaccaaggtggacaagagagtggaacccaagtcctgcgataagacccacacctgtccaccatgtcctgctccagaactgctcggcggaccttccgtgttcctgtttcctccaaagcctaaggacaccctgatgatctctcggacccctgaagtgacctgcgtggtggtggatgtgtctcacgaggatcccgaagtgaagttcaattggtacgtggacggcgtggaagtgcacaacgccaagaccaagcctagagaggaacagtacaactccacctacagagtggtgtccgtgctgaccgtgctgcaccaggattggctgaacggcaaagagtacaagtgcaaggtgtccaacaaggccctgcctgctcctatcgaaaagaccatctccaaggccaaaggtggcggaggaagccctgacattcagaaccccgatcctgccgtgtaccagctgagagactccaagtcctccgataagtctgtgtgcctgttcaccgacttcgactcccagaccaacgtgtcccagtccaaggactccgacgtgtacatcaccgataagtgcgtgctggacatgcggagcatggacttcaagtctaactccgccgtggcctggtctaacaagtccgatttcgcctgcgccaacgccttcaacaacagcattatccccgaggacacattcttcccatcacctgag

SEQ ID NO: 49 - DNA, 1320 bp, Artificial Sequence
  source: /note="Description of Artificial Sequence: Synthetic polynucleotide"
caggtgcagctggtggaatctggtggcggagttgtgcagcctggcagatccctgagactgtcttgtgccgcctccggcttcaccttctccagctacaccatgcactgggtccgacaggcccctggcaaaggattggagtgggtcaccttcatctcttacgacggcaacaacaagtactacgccgactccgtgaagggcagattcaccatctctcgggacaactccaagaacaccctgtacctgcagatgaactccctgagagccgaggacaccgccatctactactgtgctagaaccggctggctgggcccctttgattattggggacagggcaccctggtcaccgtgtcctctgcttccaccaagggaccctctgtgttccctctggctccttccagcaagtctacctctggcggaacagctgctctgggctgcctggtcaaggactactttcctgagcctgtgaccgtgtcttggaactctggcgctctgacatccggcgtgcacacctttccagctgtgctgcaatcctccggcctgtactctctgtcctccgtcgtgaccgtgccttctagctctctgggcacccagacctacatctgcaatgtgaaccacaagccttccaacaccaaggtggacaagagagtggaacccaagtcctgcgataagacccacacctgtccaccatgtcctgctccagaactgctcggcggaccttccgtgttcctgtttcctccaaagcctaaggacaccctgatgatctctcggacccctgaagtgacctgcgtggtggtggatgtgtctcacgaggatcccgaagtgaagttcaattggtacgtggacggcgtggaagtgcacaacgccaagaccaagcctagagaggaacagtacaactccacctacagagtggtgtccgtgctgaccgtgctgcaccaggattggctgaacggcaaagagtacaagtgcaaggtgtccaacaaggccctgcctgctcctatcgaaaagaccatctccaaggccaaaggtggcggaggaagcggtcctgacattcagaaccccgatcctgccgtgtaccagctgagagactccaagtcctccgataagtctgtgtgcctgttcaccgacttcgactcccagaccaacgtgtcccagtccaaggactccgacgtgtacatcaccgataagtgcgtgctggacatgcggagcatggacttcaagtctaactccgccgtggcctggtctaacaagtccgatttcgcctgcgccaacgccttcaacaacagcattatccccgaggacacattcttcccatcacctgag

SEQ ID NO: 50 - DNA, 1323 bp, Artificial Sequence
  source: /note="Description of Artificial Sequence: Synthetic polynucleotide"
caggtgcagctggtggaatctggtggcggagttgtgcagcctggcagatccctgagactgtcttgtgccgcctccggcttcaccttctccagctacaccatgcactgggtccgacaggcccctggcaaaggattggagtgggtcaccttcatctcttacgacggcaacaacaagtactacgccgactccgtgaagggcagattcaccatctctcgggacaactccaagaacaccctgtacctgcagatgaactccctgagagccgaggacaccgccatctactactgtgctagaaccggctggctgggcccctttgattattggggacagggcaccctggtcaccgtgtcctctgcttccaccaagggaccctctgtgttccctctggctccttccagcaagtctacctctggcggaacagctgctctgggctgcctggtcaaggactactttcctgagcctgtgaccgtgtcttggaactctggcgctctgacatccggcgtgcacacctttccagctgtgctgcaatcctccggcctgtactctctgtcctccgtcgtgaccgtgccttctagctctctgggcacccagacctacatctgcaatgtgaaccacaagccttccaacaccaaggtggacaagagagtggaacccaagtcctgcgataagacccacacctgtccaccatgtcctgctccagaactgctcggcggaccttccgtgttcctgtttcctccaaagcctaaggacaccctgatgatctctcggacccctgaagtgacctgcgtggtggtggatgtgtctcacgaggatcccgaagtgaagttcaattggtacgtggacggcgtggaagtgcacaacgccaagaccaagcctagagaggaacagtacaactccacctacagagtggtgtccgtgctgaccgtgctgcaccaggattggctgaacggcaaagagtacaagtgcaaggtgtccaacaaggccctgcctgctcctatcgaaaagaccatctccaaggccaaaggtggcggaggaagcggtggccctgacattcagaaccccgatcctgccgtgtaccagctgagagactccaagtcctccgataagtctgtgtgcctgttcaccgacttcgactcccagaccaacgtgtcccagtccaaggactccgacgtgtacatcaccgataagtgcgtgctggacatgcggagcatggacttcaagtctaactccgccgtggcctggtctaacaagtccgatttcgcctgcgccaacgccttcaacaacagcattatccccgaggacacattcttcccatcacctgag

SEQ ID NO: 51 - DNA, 1326 bp, Artificial Sequence
  source: /note="Description of Artificial Sequence: Synthetic polynucleotide"
caggtgcagctggtggaatctggtggcggagttgtgcagcctggcagatccctgagactgtcttgtgccgcctccggcttcaccttctccagctacaccatgcactgggtccgacaggcccctggcaaaggattggagtgggtcaccttcatctcttacgacggcaacaacaagtactacgccgactccgtgaagggcagattcaccatctctcgggacaactccaagaacaccctgtacctgcagatgaactccctgagagccgaggacaccgccatctactactgtgctagaaccggctggctgggcccctttgattattggggacagggcaccctggtcaccgtgtcctctgcttccaccaagggaccctctgtgttccctctggctccttccagcaagtctacctctggcggaacagctgctctgggctgcctggtcaaggactactttcctgagcctgtgaccgtgtcttggaactctggcgctctgacatccggcgtgcacacctttccagctgtgctgcaatcctccggcctgtactctctgtcctccgtcgtgaccgtgccttctagctctctgggcacccagacctacatctgcaatgtgaaccacaagccttccaacaccaaggtggacaagagagtggaacccaagtcctgcgataagacccacacctgtccaccatgtcctgctccagaactgctcggcggaccttccgtgttcctgtttcctccaaagcctaaggacaccctgatgatctctcggacccctgaagtgacctgcgtggtggtggatgtgtctcacgaggatcccgaagtgaagttcaattggtacgtggacggcgtggaagtgcacaacgccaagaccaagcctagagaggaacagtacaactccacctacagagtggtgtccgtgctgaccgtgctgcaccaggattggctgaacggcaaagagtacaagtgcaaggtgtccaacaaggccctgcctgctcctatcgaaaagaccatctccaaggccaaaggtggcggaggaagcggtggcggccctgacattcagaaccccgatcctgccgtgtaccagctgagagactccaagtcctccgataagtctgtgtgcctgttcaccgacttcgactcccagaccaacgtgtcccagtccaaggactccgacgtgtacatcaccgataagtgcgtgctggacatgcggagcatggacttcaagtctaactccgccgtggcctggtctaacaagtccgatttcgcctgcgccaacgccttcaacaacagcattatccccgaggacacattcttcccatcacctgag

SEQ ID NO: 52 - DNA, 1329 bp, Artificial Sequence
  source: /note="Description of Artificial Sequence: Synthetic polynucleotide"
caggtgcagctggtggaatctggtggcggagttgtgcagcctggcagatccctgagactgtcttgtgccgcctccggcttcaccttctccagctacaccatgcactgggtccgacaggcccctggcaaaggattggagtgggtcaccttcatctcttacgacggcaacaacaagtactacgccgactccgtgaagggcagattcaccatctctcgggacaactccaagaacaccctgtacctgcagatgaactccctgagagccgaggacaccgccatctactactgtgctagaaccggctggctgggcccctttgattattggggacagggcaccctggtcaccgtgtcctctgcttccaccaagggaccctctgtgttccctctggctccttccagcaagtctacctctggcggaacagctgctctgggctgcctggtcaaggactactttcctgagcctgtgaccgtgtcttggaactctggcgctctgacatccggcgtgcacacctttccagctgtgctgcaatcctccggcctgtactctctgtcctccgtcgtgaccgtgccttctagctctctgggcacccagacctacatctgcaatgtgaaccacaagccttccaacaccaaggtggacaagagagtggaacccaagtcctgcgataagacccacacctgtccaccatgtcctgctccagaactgctcggcggaccttccgtgttcctgtttcctccaaagcctaaggacaccctgatgatctctcggacccctgaagtgacctgcgtggtggtggatgtgtctcacgaggatcccgaagtgaagttcaattggtacgtggacggcgtggaagtgcacaacgccaagaccaagcctagagaggaacagtacaactccacctacagagtggtgtccgtgctgaccgtgctgcaccaggattggctgaacggcaaagagtacaagtgcaaggtgtccaacaaggccctgcctgctcctatcgaaaagaccatctccaaggccaaaggtggcggaggaagcggtggcggcggacctgacattcagaaccccgatcctgccgtgtaccagctgagagactccaagtcctccgataagtctgtgtgcctgttcaccgacttcgactcccagaccaacgtgtcccagtccaaggactccgacgtgtacatcaccgataagtgcgtgctggacatgcggagcatggacttcaagtctaactccgccgtggcctggtctaacaagtccgatttcgcctgcgccaacgccttcaacaacagcattatccccgaggacacattcttcccatcacctgag

SEQ ID NO: 53 - DNA, 1332 bp, Artificial Sequence
  source: /note="Description of Artificial Sequence: Synthetic polynucleotide"
caggtgcagctggtggaatctggtggcggagttgtgcagcctggcagatccctgagactgtcttgtgccgcctccggcttcaccttctccagctacaccatgcactgggtccgacaggcccctggcaaaggattggagtgggtcaccttcatctcttacgacggcaacaacaagtactacgccgactccgtgaagggcagattcaccatctctcgggacaactccaagaacaccctgtacctgcagatgaactccctgagagccgaggacaccgccatctactactgtgctagaaccggctggctgggcccctttgattattggggacagggcaccctggtcaccgtgtcctctgcttccaccaagggaccctctgtgttccctctggctccttccagcaagtctacctctggcggaacagctgctctgggctgcctggtcaaggactactttcctgagcctgtgaccgtgtcttggaactctggcgctctgacatccggcgtgcacacctttccagctgtgctgcaatcctccggcctgtactctctgtcctccgtcgtgaccgtgccttctagctctctgggcacccagacctacatctgcaatgtgaaccacaagccttccaacaccaaggtggacaagagagtggaacccaagtcctgcgataagacccacacctgtccaccatgtcctgctccagaactgctcggcggaccttccgtgttcctgtttcctccaaagcctaaggacaccctgatgatctctcggacccctgaagtgacctgcgtggtggtggatgtgtctcacgaggatcccgaagtgaagttcaattggtacgtggacggcgtggaagtgcacaacgccaagaccaagcctagagaggaacagtacaactccacctacagagtggtgtccgtgctgaccgtgctgcaccaggattggctgaacggcaaagagtacaagtgcaaggtgtccaacaaggccctgcctgctcctatcgaaaagaccatctccaaggccaaaggtggcggaggaagcggtggcggcggatctcctgacattcagaaccccgatcctgccgtgtaccagctgagagactccaagtcctccgataagtctgtgtgcctgttcaccgacttcgactcccagaccaacgtgtcccagtccaaggactccgacgtgtacatcaccgataagtgcgtgctggacatgcggagcatggacttcaagtctaactccgccgtggcctggtctaacaagtccgatttcgcctgcgccaacgccttcaacaacagcattatccccgaggacacattcttcccatcacctgag

SEQ ID NO: 54 - DNA, 645 bp, Artificial Sequence
  source: /note="Description of Artificial Sequence: Synthetic polynucleotide"
gagatcgtgctgacccagtctcctggcacactgtcactgtctccaggcgagagagctaccctgtcctgtagagcctctcagtccgtgggctcctcttacctggcttggtatcagcagaagcccggccaggctcctagactgttgatctacggcgccttctccagagccacaggcatccctgatagattctccggctctggctctggcaccgacttcaccctgaccatctccagactggaacccgaggacttcgccgtgtactactgtcagcagtacggctcctctccttggacctttggccagggcaccaaggtggaaatcaagcggacagtggccgctccttccgtgttcatcttcccaccttccgacgagcagctgaagtccggcacagcttctgtcgtgtgcctgctgaacaacttctaccctcgggaagccaaggtgcagtggaaggtggacaatgccctgcagtccggcaactcccaagagtctgtgaccgagcaggactccaaggacagcacctacagcctgtcctccacactgaccctgtccaaggccgactacgagaagcacaaggtgtacgcctgcgaagtgacccatcagggcctgtctagccctgtgaccaagtctttcaaccggggcgagtgc

SEQ ID NO: 55 - DNA, 1404 bp, Artificial Sequence
  source: /note="Description of Artificial Sequence: Synthetic polynucleotide"
caggtgcagctggtggaatctggtggcggagttgtgcagcctggcagatccctgagactgtcttgtgccgcctccggcttcaccttctcctcttacggaatgcactgggtccgacaggcccctggcaaaggattggagtgggtcgccttcatcagatacgacggctccaacaagtactacgccgactccgtgaagggcagattcaccatctctcgggacaactccaagaacaccctgtacctgcagatgaactccctgagagccgaggacaccgccgtgtactactgcaagacccacggctctcacgacaattggggccagggcacaatggtcaccgtgtcctctgcttccaccaagggaccctctgtgttccctctggctccttccagcaagtctacctctggcggaacagctgctctgggctgcctggtcaaggactactttcctgagcctgtgaccgtgtcttggaactctggcgctctgacatccggcgtgcacacctttccagctgtgctgcaatcctccggcctgtactctctgtcctccgtcgtgaccgtgccttctagctctctgggcacccagacctacatctgcaatgtgaaccacaagccttccaacaccaaggtggacaagagagtggaacccaagtcctgcgataagacccacacctgtccaccatgtcctgctccagaactgctcggcggaccttccgtgttcctgtttcctccaaagcctaaggacaccctgatgatctctcggacccctgaagtgacctgcgtggtggtggatgtgtctcacgaggatcccgaagtgaagttcaattggtacgtggacggcgtggaagtgcacaacgccaagaccaagcctagagaggaacagtacaactccacctacagagtggtgtccgtgctgaccgtgctgcaccaggattggctgaacggcaaagagtacaagtgcaaggtgtccaacaaggccctgcctgctcctatcgaaaagaccatctccaaggccaaagaggacctgaacaaggttttcccacctgaggtggccctgttcgagccttctgaggctgagatctctcacacccagaaagctaccctcgtgtgtctggccaccggcttctaccctgatcacgtggaactgtcttggtgggtcaacggaaaagaggtgcactccggcgtctgcaccgatcctcagcctctgaaagaacagcccgctctgaacgactccagatacgccctgtcctctcggctgagagtgtctgccaccttctggcaggaccctcggaaccactttagatgccaggtgcagttctacggcctgtccgaggctgatgagtggacccaggctagagccaagccagtgacacagatcgtgtctgccgaagcctggggcagagccgat

SEQ ID NO: 56 - DNA, 1407 bp, Artificial Sequence
  source: /note="Description of Artificial Sequence: Synthetic polynucleotide"
caggtgcagctggtggaatctggtggcggagttgtgcagcctggcagatccctgagactgtcttgtgccgcctccggcttcaccttctcctcttacggaatgcactgggtccgacaggcccctggcaaaggattggagtgggtcgccttcatcagatacgacggctccaacaagtactacgccgactccgtgaagggcagattcaccatctctcgggacaactccaagaacaccctgtacctgcagatgaactccctgagagccgaggacaccgccgtgtactactgcaagacccacggctctcacgacaattggggccagggcacaatggtcaccgtgtcctctgcttccaccaagggaccctctgtgttccctctggctccttccagcaagtctacctctggcggaacagctgctctgggctgcctggtcaaggactactttcctgagcctgtgaccgtgtcttggaactctggcgctctgacatccggcgtgcacacctttccagctgtgctgcaatcctccggcctgtactctctgtcctccgtcgtgaccgtgccttctagctctctgggcacccagacctacatctgcaatgtgaaccacaagccttccaacaccaaggtggacaagagagtggaacccaagtcctgcgataagacccacacctgtccaccatgtcctgctccagaactgctcggcggaccttccgtgttcctgtttcctccaaagcctaaggacaccctgatgatctctcggacccctgaagtgacctgcgtggtggtggatgtgtctcacgaggatcccgaagtgaagttcaattggtacgtggacggcgtggaagtgcacaacgccaagaccaagcctagagaggaacagtacaactccacctacagagtggtgtccgtgctgaccgtgctgcaccaggattggctgaacggcaaagagtacaagtgcaaggtgtccaacaaggccctgcctgctcctatcgaaaagaccatctccaaggccaaaggtgaggacctgaacaaggttttcccacctgaggtggccctgttcgagccttctgaggctgagatctctcacacccagaaagctaccctcgtgtgtctggccaccggcttctaccctgatcacgtggaactgtcttggtgggtcaacggaaaagaggtgcactccggcgtctgcaccgatcctcagcctctgaaagaacagcccgctctgaacgactccagatacgccctgtcctctcggctgagagtgtctgccaccttctggcaggaccctcggaaccactttagatgccaggtgcagttctacggcctgtccgaggctgatgagtggacccaggctagagccaagccagtgacacagatcgtgtctgccgaagcctggggcagagccgat

SEQ ID NO: 57 - DNA, 1410 bp, Artificial Sequence
  source: /note="Description of Artificial Sequence: Synthetic polynucleotide"
caggtgcagctggtggaatctggtggcggagttgtgcagcctggcagatccctgagactgtcttgtgccgcctccggcttcaccttctcctcttacggaatgcactgggtccgacaggcccctggcaaaggattggagtgggtcgccttcatcagatacgacggctccaacaagtactacgccgactccgtgaagggcagattcaccatctctcgggacaactccaagaacaccctgtacctgcagatgaactccctgagagccgaggacaccgccgtgtactactgcaagacccacggctctcacgacaattggggccagggcacaatggtcaccgtgtcctctgcttccaccaagggaccctctgtgttccctctggctccttccagcaagtctacctctggcggaacagctgctctgggctgcctggtcaaggactactttcctgagcctgtgaccgtgtcttggaactctggcgctctgacatccggcgtgcacacctttccagctgtgctgcaatcctccggcctgtactctctgtcctccgtcgtgaccgtgccttctagctctctgggcacccagacctacatctgcaatgtgaaccacaagccttccaacaccaaggtggacaagagagtggaacccaagtcctgcgataagacccacacctgtccaccatgtcctgctccagaactgctcggcggaccttccgtgttcctgtttcctccaaagcctaaggacaccctgatgatctctcggacccctgaagtgacctgcgtggtggtggatgtgtctcacgaggatcccgaagtgaagttcaattggtacgtggacggcgtggaagtgcacaacgccaagaccaagcctagagaggaacagtacaactccacctacagagtggtgtccgtgctgaccgtgctgcaccaggattggctgaacggcaaagagtacaagtgcaaggtgtccaacaaggccctgcctgctcctatcgaaaagaccatctccaaggccaaaggtggcgaggacctgaacaaggttttcccacctgaggtggccctgttcgagccttctgaggctgagatctctcacacccagaaagctaccctcgtgtgtctggccaccggcttctaccctgatcacgtggaactgtcttggtgggtcaacggaaaagaggtgcactccggcgtctgcaccgatcctcagcctctgaaagaacagcccgctctgaacgactccagatacgccctgtcctctcggctgagagtgtctgccaccttctggcaggaccctcggaaccactttagatgccaggtgcagttctacggcctgtccgaggctgatgagtggacccaggctagagccaagccagtgacacagatcgtgtctgccgaagcctggggcagagccgat

SEQ ID NO: 58 - DNA, 1413 bp, Artificial Sequence
  source: /note="Description of Artificial Sequence: Synthetic polynucleotide"
caggtgcagctggtggaatctggtggcggagttgtgcagcctggcagatccctgagactgtcttgtgccgcctccggcttcaccttctcctcttacggaatgcactgggtccgacaggcccctggcaaaggattggagtgggtcgccttcatcagatacgacggctccaacaagtactacgccgactccgtgaagggcagattcaccatctctcgggacaactccaagaacaccctgtacctgcagatgaactccctgagagccgaggacaccgccgtgtactactgcaagacccacggctctcacgacaattggggccagggcacaatggtcaccgtgtcctctgcttccaccaagggaccctctgtgttccctctggctccttccagcaagtctacctctggcggaacagctgctctgggctgcctggtcaaggactactttcctgagcctgtgaccgtgtcttggaactctggcgctctgacatccggcgtgcacacctttccagctgtgctgcaatcctccggcctgtactctctgtcctccgtcgtgaccgtgccttctagctctctgggcacccagacctacatctgcaatgtgaaccacaagccttccaacaccaaggtggacaagagagtggaacccaagtcctgcgataagacccacacctgtccaccatgtcctgctccagaactgctcggcggaccttccgtgttcctgtttcctccaaagcctaaggacaccctgatgatctctcggacccctgaagtgacctgcgtggtggtggatgtgtctcacgaggatcccgaagtgaagttcaattggtacgtggacggcgtggaagtgcacaacgccaagaccaagcctagagaggaacagtacaactccacctacagagtggtgtccgtgctgaccgtgctgcaccaggattggctgaacggcaaagagtacaagtgcaaggtgtccaacaaggccctgcctgctcctatcgaaaagaccatctccaaggccaaaggtggcggagaggacctgaacaaggttttcccacctgaggtggccctgttcgagccttctgaggctgagatctctcacacccagaaagctaccctcgtgtgtctggccaccggcttctaccctgatcacgtggaactgtcttggtgggtcaacggaaaagaggtgcactccggcgtctgcaccgatcctcagcctctgaaagaacagcccgctctgaacgactccagatacgccctgtcctctcggctgagagtgtctgccaccttctggcaggaccctcggaaccactttagatgccaggtgcagttctacggcctgtccgaggctgatgagtggacccaggctagagccaagccagtgacacagatcgtgtctgccgaagcctggggcagagccgat

SEQ ID NO: 59 - DNA, 1416 bp, Artificial Sequence
  source: /note="Description of Artificial Sequence: Synthetic polynucleotide"
caggtgcagctggtggaatctggtggcggagttgtgcagcctggcagatccctgagactgtcttgtgccgcctccggcttcaccttctcctcttacggaatgcactgggtccgacaggcccctggcaaaggattggagtgggtcgccttcatcagatacgacggctccaacaagtactacgccgactccgtgaagggcagattcaccatctctcgggacaactccaagaacaccctgtacctgcagatgaactccctgagagccgaggacaccgccgtgtactactgcaagacccacggctctcacgacaattggggccagggcacaatggtcaccgtgtcctctgcttccaccaagggaccctctgtgttccctctggctccttccagcaagtctacctctggcggaacagctgctctgggctgcctggtcaaggactactttcctgagcctgtgaccgtgtcttggaactctggcgctctgacatccggcgtgcacacctttccagctgtgctgcaatcctccggcctgtactctctgtcctccgtcgtgaccgtgccttctagctctctgggcacccagacctacatctgcaatgtgaaccacaagccttccaacaccaaggtggacaagagagtggaacccaagtcctgcgataagacccacacctgtccaccatgtcctgctccagaactgctcggcggaccttccgtgttcctgtttcctccaaagcctaaggacaccctgatgatctctcggacccctgaagtgacctgcgtggtggtggatgtgtctcacgaggatcccgaagtgaagttcaattggtacgtggacggcgtggaagtgcacaacgccaagaccaagcctagagaggaacagtacaactccacctacagagtggtgtccgtgctgaccgtgctgcaccaggattggctgaacggcaaagagtacaagtgcaaggtgtccaacaaggccctgcctgctcctatcgaaaagaccatctccaaggccaaaggtggcggaggagaggacctgaacaaggttttcccacctgaggtggccctgttcgagccttctgaggctgagatctctcacacccagaaagctaccctcgtgtgtctggccaccggcttctaccctgatcacgtggaactgtcttggtgggtcaacggaaaagaggtgcactccggcgtctgcaccgatcctcagcctctgaaagaacagcccgctctgaacgactccagatacgccctgtcctctcggctgagagtgtctgccaccttctggcaggaccctcggaaccactttagatgccaggtgcagttctacggcctgtccgaggctgatgagtggacccaggctagagccaagccagtgacacagatcgtgtctgccgaagcctggggcagagccgat

SEQ ID NO: 60 - DNA, 1419 bp, Artificial Sequence
  source: /note="Description of Artificial Sequence: Synthetic polynucleotide"
caggtgcagctggtggaatctggtggcggagttgtgcagcctggcagatccctgagactgtcttgtgccgcctccggcttcaccttctcctcttacggaatgcactgggtccgacaggcccctggcaaaggattggagtgggtcgccttcatcagatacgacggctccaacaagtactacgccgactccgtgaagggcagattcaccatctctcgggacaactccaagaacaccctgtacctgcagatgaactccctgagagccgaggacaccgccgtgtactactgcaagacccacggctctcacgacaattggggccagggcacaatggtcaccgtgtcctctgcttccaccaagggaccctctgtgttccctctggctccttccagcaagtctacctctggcggaacagctgctctgggctgcctggtcaaggactactttcctgagcctgtgaccgtgtcttggaactctggcgctctgacatccggcgtgcacacctttccagctgtgctgcaatcctccggcctgtactctctgtcctccgtcgtgaccgtgccttctagctctctgggcacccagacctacatctgcaatgtgaaccacaagccttccaacaccaaggtggacaagagagtggaacccaagtcctgcgataagacccacacctgtccaccatgtcctgctccagaactgctcggcggaccttccgtgttcctgtttcctccaaagcctaaggacaccctgatgatctctcggacccctgaagtgacctgcgtggtggtggatgtgtctcacgaggatcccgaagtgaagttcaattggtacgtggacggcgtggaagtgcacaacgccaagaccaagcctagagaggaacagtacaactccacctacagagtggtgtccgtgctgaccgtgctgcaccaggattggctgaacggcaaagagtacaagtgcaaggtgtccaacaaggccctgcctgctcctatcgaaaagaccatctccaaggccaaaggtggcggaggaagcgaggacctgaacaaggttttcccacctgaggtggccctgttcgagccttctgaggctgagatctctcacacccagaaagctaccctcgtgtgtctggccaccggcttctaccctgatcacgtggaactgtcttggtgggtcaacggaaaagaggtgcactccggcgtctgcaccgatcctcagcctctgaaagaacagcccgctctgaacgactccagatacgccctgtcctctcggctgagagtgtctgccaccttctggcaggaccctcggaaccactttagatgccaggtgcagttctacggcctgtccgaggctgatgagtggacccaggctagagccaagccagtgacacagatcgtgtctgccgaagcctggggcagagccgat

SEQ ID NO: 61 - DNA, 1422 bp, Artificial Sequence
  source: /note="Description of Artificial Sequence: Synthetic polynucleotide"
caggtgcagctggtggaatctggtggcggagttgtgcagcctggcagatccctgagactgtcttgtgccgcctccggcttcaccttctcctcttacggaatgcactgggtccgacaggcccctggcaaaggattggagtgggtcgccttcatcagatacgacggctccaacaagtactacgccgactccgtgaagggcagattcaccatctctcgggacaactccaagaacaccctgtacctgcagatgaactccctgagagccgaggacaccgccgtgtactactgcaagacccacggctctcacgacaattggggccagggcacaatggtcaccgtgtcctctgcttccaccaagggaccctctgtgttccctctggctccttccagcaagtctacctctggcggaacagctgctctgggctgcctggtcaaggactactttcctgagcctgtgaccgtgtcttggaactctggcgctctgacatccggcgtgcacacctttccagctgtgctgcaatcctccggcctgtactctctgtcctccgtcgtgaccgtgccttctagctctctgggcacccagacctacatctgcaatgtgaaccacaagccttccaacaccaaggtggacaagagagtggaacccaagtcctgcgataagacccacacctgtccaccatgtcctgctccagaactgctcggcggaccttccgtgttcctgtttcctccaaagcctaaggacaccctgatgatctctcggacccctgaagtgacctgcgtggtggtggatgtgtctcacgaggatcccgaagtgaagttcaattggtacgtggacggcgtggaagtgcacaacgccaagaccaagcctagagaggaacagtacaactccacctacagagtggtgtccgtgctgaccgtgctgcaccaggattggctgaacggcaaagagtacaagtgcaaggtgtccaacaaggccctgcctgctcctatcgaaaagaccatctccaaggccaaaggtggcggaggaagcggtgaggacctgaacaaggttttcccacctgaggtggccctgttcgagccttctgaggctgagatctctcacacccagaaagctaccctcgtgtgtctggccaccggcttctaccctgatcacgtggaactgtcttggtgggtcaacggaaaagaggtgcactccggcgtctgcaccgatcctcagcctctgaaagaacagcccgctctgaacgactccagatacgccctgtcctctcggctgagagtgtctgccaccttctggcaggaccctcggaaccactttagatgccaggtgcagttctacggcctgtccgaggctgatgagtggacccaggctagagccaagccagtgacacagatcgtgtctgccgaagcctggggcagagccgat

SEQ ID NO: 62 - DNA, 1425 bp, Artificial Sequence
  source: /note="Description of Artificial Sequence: Synthetic polynucleotide"
caggtgcagctggtggaatctggtggcggagttgtgcagcctggcagatccctgagactgtcttgtgccgcctccggcttcaccttctcctcttacggaatgcactgggtccgacaggcccctggcaaaggattggagtgggtcgccttcatcagatacgacggctccaacaagtactacgccgactccgtgaagggcagattcaccatctctcgggacaactccaagaacaccctgtacctgcagatgaactccctgagagccgaggacaccgccgtgtactactgcaagacccacggctctcacgacaattggggccagggcacaatggtcaccgtgtcctctgcttccaccaagggaccctctgtgttccctctggctccttccagcaagtctacctctggcggaacagctgctctgggctgcctggtcaaggactactttcctgagcctgtgaccgtgtcttggaactctggcgctctgacatccggcgtgcacacctttccagctgtgctgcaatcctccggcctgtactctctgtcctccgtcgtgaccgtgccttctagctctctgggcacccagacctacatctgcaatgtgaaccacaagccttccaacaccaaggtggacaagagagtggaacccaagtcctgcgataagacccacacctgtccaccatgtcctgctccagaactgctcggcggaccttccgtgttcctgtttcctccaaagcctaaggacaccctgatgatctctcggacccctgaagtgacctgcgtggtggtggatgtgtctcacgaggatcccgaagtgaagttcaattggtacgtggacggcgtggaagtgcacaacgccaagaccaagcctagagaggaacagtacaactccacctacagagtggtgtccgtgctgaccgtgctgcaccaggattggctgaacggcaaagagtacaagtgcaaggtgtccaacaaggccctgcctgctcctatcgaaaagaccatctccaaggccaaaggtggcggaggaagcggtggcgaggacctgaacaaggttttcccacctgaggtggccctgttcgagccttctgaggctgagatctctcacacccagaaagctaccctcgtgtgtctggccaccggcttctaccctgatcacgtggaactgtcttggtgggtcaacggaaaagaggtgcactccggcgtctgcaccgatcctcagcctctgaaagaacagcccgctctgaacgactccagatacgccctgtcctctcggctgagagtgtctgccaccttctggcaggaccctcggaaccactttagatgccaggtgcagttctacggcctgtccgaggctgatgagtggacccaggctagagccaagccagtgacacagatcgtgtctgccgaagcctggggcagagccgat

SEQ ID NO: 63 - DNA, 1428 bp, Artificial Sequence
  source: /note="Description of Artificial Sequence: Synthetic polynucleotide"
caggtgcagctggtggaatctggtggcggagttgtgcagcctggcagatccctgagactgtcttgtgccgcctccggcttcaccttctcctcttacggaatgcactgggtccgacaggcccctggcaaaggattggagtgggtcgccttcatcagatacgacggctccaacaagtactacgccgactccgtgaagggcagattcaccatctctcgggacaactccaagaacaccctgtacctgcagatgaactccctgagagccgaggacaccgccgtgtactactgcaagacccacggctctcacgacaattggggccagggcacaatggtcaccgtgtcctctgcttccaccaagggaccctctgtgttccctctggctccttccagcaagtctacctctggcggaacagctgctctgggctgcctggtcaaggactactttcctgagcctgtgaccgtgtcttggaactctggcgctctgacatccggcgtgcacacctttccagctgtgctgcaatcctccggcctgtactctctgtcctccgtcgtgaccgtgccttctagctctctgggcacccagacctacatctgcaatgtgaaccacaagccttccaacaccaaggtggacaagagagtggaacccaagtcctgcgataagacccacacctgtccaccatgtcctgctccagaactgctcggcggaccttccgtgttcctgtttcctccaaagcctaaggacaccctgatgatctctcggacccctgaagtgacctgcgtggtggtggatgtgtctcacgaggatcccgaagtgaagttcaattggtacgtggacggcgtggaagtgcacaacgccaagaccaagcctagagaggaacagtacaactccacctacagagtggtgtccgtgctgaccgtgctgcaccaggattggctgaacggcaaagagtacaagtgcaaggtgtccaacaaggccctgcctgctcctatcgaaaagaccatctccaaggccaaaggtggcggaggaagcggtggcggcgaggacctgaacaaggttttcccacctgaggtggccctgttcgagccttctgaggctgagatctctcacacccagaaagctaccctcgtgtgtctggccaccggcttctaccctgatcacgtggaactgtcttggtgggtcaacggaaaagaggtgcactccggcgtctgcaccgatcctcagcctctgaaagaacagcccgctctgaacgactccagatacgccctgtcctctcggctgagagtgtctgccaccttctggcaggaccctcggaaccactttagatgccaggtgcagttctacggcctgtccgaggctgatgagtggacccaggctagagccaagccagtgacacagatcgtgtctgccgaagcctggggcagagccgat

SEQ ID NO: 64 - DNA, 1431 bp, Artificial Sequence
  source: /note="Description of Artificial Sequence: Synthetic polynucleotide"
caggtgcagctggtggaatctggtggcggagttgtgcagcctggcagatccctgagactgtcttgtgccgcctccggcttcaccttctcctcttacggaatgcactgggtccgacaggcccctggcaaaggattggagtgggtcgccttcatcagatacgacggctccaacaagtactacgccgactccgtgaagggcagattcaccatctctcgggacaactccaagaacaccctgtacctgcagatgaactccctgagagccgaggacaccgccgtgtactactgcaagacccacggctctcacgacaattggggccagggcacaatggtcaccgtgtcctctgcttccaccaagggaccctctgtgttccctctggctccttccagcaagtctacctctggcggaacagctgctctgggctgcctggtcaaggactactttcctgagcctgtgaccgtgtcttggaactctggcgctctgacatccggcgtgcacacctttccagctgtgctgcaatcctccggcctgtactctctgtcctccgtcgtgaccgtgccttctagctctctgggcacccagacctacatctgcaatgtgaaccacaagccttccaacaccaaggtggacaagagagtggaacccaagtcctgcgataagacccacacctgtccaccatgtcctgctccagaactgctcggcggaccttccgtgttcctgtttcctccaaagcctaaggacaccctgatgatctctcggacccctgaagtgacctgcgtggtggtggatgtgtctcacgaggatcccgaagtgaagttcaattggtacgtggacggcgtggaagtgcacaacgccaagaccaagcctagagaggaacagtacaactccacctacagagtggtgtccgtgctgaccgtgctgcaccaggattggctgaacggcaaagagtacaagtgcaaggtgtccaacaaggccctgcctgctcctatcgaaaagaccatctccaaggccaaaggtggcggaggaagcggtggcggcggagaggacctgaacaaggttttcccacctgaggtggccctgttcgagccttctgaggctgagatctctcacacccagaaagctaccctcgtgtgtctggccaccggcttctaccctgatcacgtggaactgtcttggtgggtcaacggaaaagaggtgcactccggcgtctgcaccgatcctcagcctctgaaagaacagcccgctctgaacgactccagatacgccctgtcctctcggctgagagtgtctgccaccttctggcaggaccctcggaaccactttagatgccaggtgcagttctacggcctgtccgaggctgatgagtggacccaggctagagccaagccagtgacacagatcgtgtctgccgaagcctggggcagagccgat

SEQ ID NO: 65 - DNA, 1434 bp, Artificial Sequence
  source: /note="Description of Artificial Sequence: Synthetic polynucleotide"
caggtgcagctggtggaatctggtggcggagttgtgcagcctggcagatccctgagactgtcttgtgccgcctccggcttcaccttctcctcttacggaatgcactgggtccgacaggcccctggcaaaggattggagtgggtcgccttcatcagatacgacggctccaacaagtactacgccgactccgtgaagggcagattcaccatctctcgggacaactccaagaacaccctgtacctgcagatgaactccctgagagccgaggacaccgccgtgtactactgcaagacccacggctctcacgacaattggggccagggcacaatggtcaccgtgtcctctgcttccaccaagggaccctctgtgttccctctggctccttccagcaagtctacctctggcggaacagctgctctgggctgcctggtcaaggactactttcctgagcctgtgaccgtgtcttggaactctggcgctctgacatccggcgtgcacacctttccagctgtgctgcaatcctccggcctgtactctctgtcctccgtcgtgaccgtgccttctagctctctgggcacccagacctacatctgcaatgtgaaccacaagccttccaacaccaaggtggacaagagagtggaacccaagtcctgcgataagacccacacctgtccaccatgtcctgctccagaactgctcggcggaccttccgtgttcctgtttcctccaaagcctaaggacaccctgatgatctctcggacccctgaagtgacctgcgtggtggtggatgtgtctcacgaggatcccgaagtgaagttcaattggtacgtggacggcgtggaagtgcacaacgccaagaccaagcctagagaggaacagtacaactccacctacagagtggtgtccgtgctgaccgtgctgcaccaggattggctgaacggcaaagagtacaagtgcaaggtgtccaacaaggccctgcctgctcctatcgaaaagaccatctccaaggccaaaggtggcggaggaagcggtggcggcggatctgaggacctgaacaaggttttcccacctgaggtggccctgttcgagccttctgaggctgagatctctcacacccagaaagctaccctcgtgtgtctggccaccggcttctaccctgatcacgtggaactgtcttggtgggtcaacggaaaagaggtgcactccggcgtctgcaccgatcctcagcctctgaaagaacagcccgctctgaacgactccagatacgccctgtcctctcggctgagagtgtctgccaccttctggcaggaccctcggaaccactttagatgccaggtgcagttctacggcctgtccgaggctgatgagtggacccaggctagagccaagccagtgacacagatcgtgtctgccgaagcctggggcagagccgat

SEQ ID NO: 66 - DNA, 651 bp, Artificial Sequence
  source: /note="Description of Artificial Sequence: Synthetic polynucleotide"
cagtccgtgttgacccagcctccttctgtttctggcgctcctggccagagagtgaccatctcttgctccggctctcggtccaacatcggctccaataccgtgaagtggtatcagcagctgcccggcacagctcccaaactgctgatctactacaacgaccagcggccttctggcgtgcccgatagattctctggctccaagtctggcacctctgccagcctggctattaccggactgcaggctgaggacgaggccgactactactgccagtcttacgaccggtacacccatcctgctctgctgtttggcaccggcaccaaagtgacagtgctgggccagcctaaggccaatcctaccgtgacactgttccctccatcctccgaagaactgcaggccaacaaggctaccctcgtgtgcctgatctccgacttttaccctggcgctgtgaccgtggcctggaaggctgatggatctcctgtgaaggctggcgtggaaaccaccaagccttccaagcagtccaacaacaaatacgccgcctcctcctacctgtctctgacccctgaacagtggaagtcccaccggtcctacagctgccaagtgacccatgagggctccaccgtggaaaagaccgtggctcctaccgagtgctcc

SEQ ID NO: 67 - DNA, 708 bp, Artificial Sequence
  source: /note="Description of Artificial Sequence: Synthetic polynucleotide"
accatcaagccttgtcctccatgcaagtgccccgctcctaatctgctcggaggcccttccgtgttcatcttcccacctaagatcaaggacgtgctgatgatctccctgtctcctatcgtgacctgcgtggtggtggacgtgtccgaggatgatcctgacgtgcagatcagttggttcgtgaacaacgtggaagtgcacaccgctcagacccagacacacagagaggactacaacagcaccctgagagtggtgtctgccctgcctatccagcaccaggattggatgtccggcaaagaattcaagtgcaaagtgaacaacaaggacctgcctgctccaatcgagcggaccatctccaagcctaagcctaacatccagaatcctgagcctgccgtgtaccagctgaaggaccctagatctcaggactctaccctgtgcctgttcaccgacttcgactcccagatcaacgtgcccaagaccatggaatccggcaccttcatcaccgataagtgcgtgctggacatgaaggccatggactccaagtccaacggcgctatcgcctggtccaaccagaccagcttcacatgccaggacatcttcaaagagacaaacgccacctatccttccagcgacgtgccctgtgatgctaccctgaccgagaagtccttcgagacagacatgaacctgaacttccagaacctgtcctgatga

SEQ ID NO: 68 - DNA, 711 bp, Artificial Sequence
  source: /note="Description of Artificial Sequence: Synthetic polynucleotide"
accatcaagccttgtcctccatgcaagtgccccgctcctaatctgctcggaggcccttccgtgttcatcttcccacctaagatcaaggacgtgctgatgatctccctgtctcctatcgtgacctgcgtggtggtggacgtgtccgaggatgatcctgacgtgcagatcagttggttcgtgaacaacgtggaagtgcacaccgctcagacccagacacacagagaggactacaacagcaccctgagagtggtgtctgccctgcctatccagcaccaggattggatgtccggcaaagaattcaagtgcaaagtgaacaacaaggacctgcctgctccaatcgagcggaccatctccaagcctggtaagcctaacatccagaatcctgagcctgccgtgtaccagctgaaggaccctagatctcaggactctaccctgtgcctgttcaccgacttcgactcccagatcaacgtgcccaagaccatggaatccggcaccttcatcaccgataagtgcgtgctggacatgaaggccatggactccaagtccaacggcgctatcgcctggtccaaccagaccagcttcacatgccaggacatcttcaaagagacaaacgccacctatccttccagcgacgtgccctgtgatgctaccctgaccgagaagtccttcgagacagacatgaacctgaacttccagaacctgtcctgatga

SEQ ID NO: 69 - DNA, 675 bp, Artificial Sequence
  source: /note="Description of Artificial Sequence: Synthetic polynucleotide"
accatcaagccttgtcctccatgcaagtgccccgctcctaatctgctcggaggcccttccgtgttcatcttcccacctaagatcaaggacgtgctgatgatctccctgtctcctatcgtgacctgcgtggtggtggacgtgtccgaggatgatcctgacgtgcagatcagttggttcgtgaacaacgtggaagtgcacaccgctcagacccagacacacagagaggactacaacagcaccctgagagtggtgtctgccctgcctatccagcaccaggattggatgtccggcaaagaattcaagtgcaaagtgaacaacaaggacctgcctgctccaatcgagcggaccatctccaagcctggtggcgcttccaccaagggaccctctgtgttccctctggctccttccagcaagtctacctctggcggaacagctgctctgggctgcctggtcaaggactactttcctgagcctgtgaccgtgtcttggaactctggcgctctgacatccggcgtgcacacctttccagctgtgctgcaatcctccggcctgtactctctgtcctccgtcgtgaccgtgccttctagctctctgggcacccagacctacatctgcaatgtgaaccacaagccttccaacaccaaggtggacaagagagtggaacccaagtcctgc

SEQ ID NO: 70 - DNA, 717 bp, Artificial Sequence
  source: /note="Description of Artificial Sequence: Synthetic polynucleotide"
accatcaagccttgtcctccatgcaagtgccccgctcctaatctgctcggaggcccttccgtgttcatcttcccacctaagatcaaggacgtgctgatgatctccctgtctcctatcgtgacctgcgtggtggtggacgtgtccgaggatgatcctgacgtgcagatcagttggttcgtgaacaacgtggaagtgcacaccgctcagacccagacacacagagaggactacaacagcaccctgagagtggtgtctgccctgcctatccagcaccaggattggatgtccggcaaagaattcaagtgcaaagtgaacaacaaggacctgcctgctccaatcgagcggaccatctccaagcctggtggcggaaagcctaacatccagaatcctgagcctgccgtgtaccagctgaaggaccctagatctcaggactctaccctgtgcctgttcaccgacttcgactcccagatcaacgtgcccaagaccatggaatccggcaccttcatcaccgataagtgcgtgctggacatgaaggccatggactccaagtccaacggcgctatcgcctggtccaaccagaccagcttcacatgccaggacatcttcaaagagacaaacgccacctatccttccagcgacgtgccctgtgatgctaccctgaccgagaagtccttcgagacagacatgaacctgaacttccagaacctgtcctgatga

SEQ ID NO: 71 - DNA, 720 bp, Artificial Sequence
  source: /note="Description of Artificial Sequence: Synthetic polynucleotide"
accatcaagccttgtcctccatgcaagtgccccgctcctaatctgctcggaggcccttccgtgttcatcttcccacctaagatcaaggacgtgctgatgatctccctgtctcctatcgtgacctgcgtggtggtggacgtgtccgaggatgatcctgacgtgcagatcagttggttcgtgaacaacgtggaagtgcacaccgctcagacccagacacacagagaggactacaacagcaccctgagagtggtgtctgccctgcctatccagcaccaggattggatgtccggcaaagaattcaagtgcaaagtgaacaacaaggacctgcctgctccaatcgagcggaccatctccaagcctggtggcggaggaaagcctaacatccagaatcctgagcctgccgtgtaccagctgaaggaccctagatctcaggactctaccctgtgcctgttcaccgacttcgactcccagatcaacgtgcccaagaccatggaatccggcaccttcatcaccgataagtgcgtgctggacatgaaggccatggactccaagtccaacggcgctatcgcctggtccaaccagaccagcttcacatgccaggacatcttcaaagagacaaacgccacctatccttccagcgacgtgccctgtgatgctaccctgaccgagaagtccttcgagacagacatgaacctgaacttccagaacctgtcctgatga

SEQ ID NO: 72 - DNA, 723 bp, Artificial Sequence
  source: /note="Description of Artificial Sequence: Synthetic polynucleotide"
accatcaagccttgtcctccatgcaagtgccccgctcctaatctgctcggaggcccttccgtgttcatcttcccacctaagatcaaggacgtgctgatgatctccctgtctcctatcgtgacctgcgtggtggtggacgtgtccgaggatgatcctgacgtgcagatcagttggttcgtgaacaacgtggaagtgcacaccgctcagacccagacacacagagaggactacaacagcaccctgagagtggtgtctgccctgcctatccagcaccaggattggatgtccggcaaagaattcaagtgcaaagtgaacaacaaggacctgcctgctccaatcgagcggaccatctccaagcctggtggcggaggaagcaagcctaacatccagaatcctgagcctgccgtgtaccagctgaaggaccctagatctcaggactctaccctgtgcctgttcaccgacttcgactcccagatcaacgtgcccaagaccatggaatccggcaccttcatcaccgataagtgcgtgctggacatgaaggccatggactccaagtccaacggcgctatcgcctggtccaaccagaccagcttcacatgccaggacatcttcaaagagacaaacgccacctatccttccagcgacgtgccctgtgatgctaccctgaccgagaagtccttcgagacagacatgaacctgaacttccagaacctgtcctgatga

SEQ ID NO: 73 - DNA, 726 bp, Artificial Sequence
  source: /note="Description of Artificial Sequence: Synthetic polynucleotide"
accatcaagccttgtcctccatgcaagtgccccgctcctaatctgctcggaggcccttccgtgttcatcttcccacctaagatcaaggacgtgctgatgatctccctgtctcctatcgtgacctgcgtggtggtggacgtgtccgaggatgatcctgacgtgcagatcagttggttcgtgaacaacgtggaagtgcacaccgctcagacccagacacacagagaggactacaacagcaccctgagagtggtgtctgccctgcctatccagcaccaggattggatgtccggcaaagaattcaagtgcaaagtgaacaacaaggacctgcctgctccaatcgagcggaccatctccaagcctggtggcggaggaagcggtaagcctaacatccagaatcctgagcctgccgtgtaccagctgaaggaccctagatctcaggactctaccctgtgcctgttcaccgacttcgactcccagatcaacgtgcccaagaccatggaatccggcaccttcatcaccgataagtgcgtgctggacatgaaggccatggactccaagtccaacggcgctatcgcctggtccaaccagaccagcttcacatgccaggacatcttcaaagagacaaacgccacctatccttccagcgacgtgccctgtgatgctaccctgaccgagaagtccttcgagacagacatgaacctgaacttccagaacctgtcctgatga

SEQ ID NO: 74 - DNA, 729 bp, Artificial Sequence
  source: /note="Description of Artificial Sequence: Synthetic polynucleotide"
accatcaagccttgtcctccatgcaagtgccccgctcctaatctgctcggaggcccttccgtgttcatcttcccacctaagatcaaggacgtgctgatgatctccctgtctcctatcgtgacctgcgtggtggtggacgtgtccgaggatgatcctgacgtgcagatcagttggttcgtgaacaacgtggaagtgcacaccgctcagacccagacacacagagaggactacaacagcaccctgagagtggtgtctgccctgcctatccagcaccaggattggatgtccggcaaagaattcaagtgcaaagtgaacaacaaggacctgcctgctccaatcgagcggaccatctccaagcctggtggcggaggaagcggtggcaagcctaacatccagaatcctgagcctgccgtgtaccagctgaaggaccctagatctcaggactctaccctgtgcctgttcaccgacttcgactcccagatcaacgtgcccaagaccatggaatccggcaccttcatcaccgataagtgcgtgctggacatgaaggccatggactccaagtccaacggcgctatcgcctggtccaaccagaccagcttcacatgccaggacatcttcaaagagacaaacgccacctatccttccagcgacgtgccctgtgatgctaccctgaccgagaagtccttcgagacagacatgaacctgaacttccagaacctgtcctgatga

SEQ ID NO: 75 - DNA, 732 bp, Artificial Sequence
  source: /note="Description of Artificial Sequence: Synthetic polynucleotide"
accatcaagccttgtcctccatgcaagtgccccgctcctaatctgctcggaggcccttccgtgttcatcttcccacctaagatcaaggacgtgctgatgatctccctgtctcctatcgtgacctgcgtggtggtggacgtgtccgaggatgatcctgacgtgcagatcagttggttcgtgaacaacgtggaagtgcacaccgctcagacccagacacacagagaggactacaacagcaccctgagagtggtgtctgccctgcctatccagcaccaggattggatgtccggcaaagaattcaagtgcaaagtgaacaacaaggacctgcctgctccaatcgagcggaccatctccaagcctggtggcggaggaagcggtggcggcaagcctaacatccagaatcctgagcctgccgtgtaccagctgaaggaccctagatctcaggactctaccctgtgcctgttcaccgacttcgactcccagatcaacgtgcccaagaccatggaatccggcaccttcatcaccgataagtgcgtgctggacatgaaggccatggactccaagtccaacggcgctatcgcctggtccaaccagaccagcttcacatgccaggacatcttcaaagagacaaacgccacctatccttccagcgacgtgccctgtgatgctaccctgaccgagaagtccttcgagacagacatgaacctgaacttccagaacctgtcctgatga

SEQ ID NO: 76 - DNA, 735 bp, Artificial Sequence
  source: /note="Description of Artificial Sequence: Synthetic polynucleotide"
accatcaagccttgtcctccatgcaagtgccccgctcctaatctgctcggaggcccttccgtgttcatcttcccacctaagatcaaggacgtgctgatgatctccctgtctcctatcgtgacctgcgtggtggtggacgtgtccgaggatgatcctgacgtgcagatcagttggttcgtgaacaacgtggaagtgcacaccgctcagacccagacacacagagaggactacaacagcaccctgagagtggtgtctgccctgcctatccagcaccaggattggatgtccggcaaagaattcaagtgcaaagtgaacaacaaggacctgcctgctccaatcgagcggaccatctccaagcctggtggcggaggaagcggtggcggcggaaagcctaacatccagaatcctgagcctgccgtgtaccagctgaaggaccctagatctcaggactctaccctgtgcctgttcaccgacttcgactcccagatcaacgtgcccaagaccatggaatccggcaccttcatcaccgataagtgcgtgctggacatgaaggccatggactccaagtccaacggcgctatcgcctggtccaaccagaccagcttcacatgccaggacatcttcaaagagacaaacgccacctatccttccagcgacgtgccctgtgatgctaccctgaccgagaagtccttcgagacagacatgaacctgaacttccagaacctgtcctgatga

SEQ ID NO: 77 - DNA, 738 bp, Artificial Sequence
  source: /note="Description of Artificial Sequence: Synthetic polynucleotide"
accatcaagccttgtcctccatgcaagtgccccgctcctaatctgctcggaggcccttccgtgttcatcttcccacctaagatcaaggacgtgctgatgatctccctgtctcctatcgtgacctgcgtggtggtggacgtgtccgaggatgatcctgacgtgcagatcagttggttcgtgaacaacgtggaagtgcacaccgctcagacccagacacacagagaggactacaacagcaccctgagagtggtgtctgccctgcctatccagcaccaggattggatgtccggcaaagaattcaagtgcaaagtgaacaacaaggacctgcctgctccaatcgagcggaccatctccaagcctggtggcggaggaagcggtggcggcggatctaagcctaacatccagaatcctgagcctgccgtgtaccagctgaaggaccctagatctcaggactctaccctgtgcctgttcaccgacttcgactcccagatcaacgtgcccaagaccatggaatccggcaccttcatcaccgataagtgcgtgctggacatgaaggccatggactccaagtccaacggcgctatcgcctggtccaaccagaccagcttcacatgccaggacatcttcaaagagacaaacgccacctatccttccagcgacgtgccctgtgatgctaccctgaccgagaagtccttcgagacagacatgaacctgaacttccagaacctgtcctgatga

SEQ ID NO: 78 - DNA, 1167 bp, Artificial Sequence
  source: /note="Description of Artificial Sequence: Synthetic polynucleotide"
accatcaagccttgtcctccatgcaagtgccccgctcctaatctgctcggaggcccttccgtgttcatcttcccacctaagatcaaggacgtgctgatgatctccctgtctcctatcgtgacctgcgtggtggtggacgtgtccgaggatgatcctgacgtgcagatcagttggttcgtgaacaacgtggaagtgcacaccgctcagacccagacacacagagaggactacaacagcaccctgagagtggtgtctgccctgcctatccagcaccaggattggatgtccggcaaagaattcaagtgcaaagtgaacaacaaggacctgcctgctccaatcgagcggaccatctccaagcctgtggtggaagatctgcggaacgtgacccctcctaaggtgtccctgttcgagccttccaaggccgagatcgccaacaagcagaaagctaccctcgtgtgcctggccagaggcttctttcctgaccacgtggaactgtcttggtgggtcaacggcaaagaggtgcactccggcgtctgtaccgatcctcaggcctacaaagagtccaactactcctacagcctgtcctctcggctgagagtgtctgccaccttctggcacaaccctcggaaccacttcagatgccaggtgcagtttcacggcctgtccgaagaggacaagtggcctgagggatcccctaagcctgtgacacagaacatctctgccgaggcctggggtagagctgatggtggcggaggatctggcggaggtggaagcggcggaggcggatcttctcatctggaacagctgctgatggacctgcaagagctgctgtcccggatggaaaactaccggaacctgaagctgccccggatgctgaccgctaagttcgctctgcctaagcaggccaccgagctgaaggatctgcagtgcctggaagatgagctgggccctctgagacacgtgctggatctgacccagtccaagtcctttcagctcgaggacgccgagaacttcatctccaacatcagagtgaccgtggtcaagctgaagggctccgacaacaccttcgagtgccagttcgacgatgagtccgctacagtggtggacttcctgcggagatggatcgccttctgccagtccatcatctccacctctccacagtgatga

SEQ ID NO: 79 - DNA, 1170 bp, Artificial Sequence
  source: /note="Description of Artificial Sequence: Synthetic polynucleotide"
accatcaagccttgtcctccatgcaagtgccccgctcctaatctgctcggaggcccttccgtgttcatcttcccacctaagatcaaggacgtgctgatgatctccctgtctcctatcgtgacctgcgtggtggtggacgtgtccgaggatgatcctgacgtgcagatcagttggttcgtgaacaacgtggaagtgcacaccgctcagacccagacacacagagaggactacaacagcaccctgagagtggtgtctgccctgcctatccagcaccaggattggatgtccggcaaagaattcaagtgcaaagtgaacaacaaggacctgcctgctccaatcgagcggaccatctccaagcctggtgtggtggaagatctgcggaacgtgacccctcctaaggtgtccctgttcgagccttccaaggccgagatcgccaacaagcagaaagctaccctcgtgtgcctggccagaggcttctttcctgaccacgtggaactgtcttggtgggtcaacggcaaagaggtgcactccggcgtctgtaccgatcctcaggcctacaaagagtccaactactcctacagcctgtcctctcggctgagagtgtctgccaccttctggcacaaccctcggaaccacttcagatgccaggtgcagtttcacggcctgtccgaagaggacaagtggcctgagggatcccctaagcctgtgacacagaacatctctgccgaggcctggggtagagctgatggtggcggaggatctggcggaggtggaagcggcggaggcggatcttctcatctggaacagctgctgatggacctgcaagagctgctgtcccggatggaaaactaccggaacctgaagctgccccggatgctgaccgctaagttcgctctgcctaagcaggccaccgagctgaaggatctgcagtgcctggaagatgagctgggccctctgagacacgtgctggatctgacccagtccaagtcctttcagctcgaggacgccgagaacttcatctccaacatcagagtgaccgtggtcaagctgaagggctccgacaacaccttcgagtgccagttcgacgatgagtccgctacagtggtggacttcctgcggagatggatcgccttctgccagtccatcatctccacctctccacagtgatga

SEQ ID NO: 80 - DNA, 1173 bp, Artificial Sequence
  source: /note="Description of Artificial Sequence: Synthetic polynucleotide"
accatcaagccttgtcctccatgcaagtgccccgctcctaatctgctcggaggcccttccgtgttcatcttcccacctaagatcaaggacgtgctgatgatctccctgtctcctatcgtgacctgcgtggtggtggacgtgtccgaggatgatcctgacgtgcagatcagttggttcgtgaacaacgtggaagtgcacaccgctcagacccagacacacagagaggactacaacagcaccctgagagtggtgtctgccctgcctatccagcaccaggattggatgtccggcaaagaattcaagtgcaaagtgaacaacaaggacctgcctgctccaatcgagcggaccatctccaagcctggtggcgtggtggaagatctgcggaacgtgacccctcctaaggtgtccctgttcgagccttccaaggccgagatcgccaacaagcagaaagctaccctcgtgtgcctggccagaggcttctttcctgaccacgtggaactgtcttggtgggtcaacggcaaagaggtgcactccggcgtctgtaccgatcctcaggcctacaaagagtccaactactcctacagcctgtcctctcggctgagagtgtctgccaccttctggcacaaccctcggaaccacttcagatgccaggtgcagtttcacggcctgtccgaagaggacaagtggcctgagggatcccctaagcctgtgacacagaacatctctgccgaggcctggggtagagctgatggtggcggaggatctggcggaggtggaagcggcggaggcggatcttctcatctggaacagctgctgatggacctgcaagagctgctgtcccggatggaaaactaccggaacctgaagctgccccggatgctgaccgctaagttcgctctgcctaagcaggccaccgagctgaaggatctgcagtgcctggaagatgagctgggccctctgagacacgtgctggatctgacccagtccaagtcctttcagctcgaggacgccgagaacttcatctccaacatcagagtgaccgtggtcaagctgaagggctccgacaacaccttcgagtgccagttcgacgatgagtccgctacagtggtggacttcctgcggagatggatcgccttctgccagtccatcatctccacctctccacagtgatga

SEQ ID NO: 81 - DNA, 1176 bp, Artificial Sequence
  source: /note="Description of Artificial Sequence: Synthetic polynucleotide"
accatcaagccttgtcctccatgcaagtgccccgctcctaatctgctcggaggcccttccgtgttcatcttcccacctaagatcaaggacgtgctgatgatctccctgtctcctatcgtgacctgcgtggtggtggacgtgtccgaggatgatcctgacgtgcagatcagttggttcgtgaacaacgtggaagtgcacaccgctcagacccagacacacagagaggactacaacagcaccctgagagtggtgtctgccctgcctatccagcaccaggattggatgtccggcaaagaattcaagtgcaaagtgaacaacaaggacctgcctgctccaatcgagcggaccatctccaagcctggtggcggagtggtggaagatctgcggaacgtgacccctcctaaggtgtccctgttcgagccttccaaggccgagatcgccaacaagcagaaagctaccctcgtgtgcctggccagaggcttctttcctgaccacgtggaactgtcttggtgggtcaacggcaaagaggtgcactccggcgtctgtaccgatcctcaggcctacaaagagtccaactactcctacagcctgtcctctcggctgagagtgtctgccaccttctggcacaaccctcggaaccacttcagatgccaggtgcagtttcacggcctgtccgaagaggacaagtggcctgagggatcccctaagcctgtgacacagaacatctctgccgaggcctggggtagagctgatggtggcggaggatctggcggaggtggaagcggcggaggcggatcttctcatctggaacagctgctgatggacctgcaagagctgctgtcccggatggaaaactaccggaacctgaagctgccccggatgctgaccgctaagttcgctctgcctaagcaggccaccgagctgaaggatctgcagtgcctggaagatgagctgggccctctgagacacgtgctggatctgacccagtccaagtcctttcagctcgaggacgccgagaacttcatctccaacatcagagtgaccgtggtcaagctgaagggctccgacaacaccttcgagtgccagttcgacgatgagtccgctacagtggtggacttcctgcggagatggatcgccttctgccagtccatcatctccacctctccacagtgatga

SEQ ID NO: 82 - DNA, 1179 bp, Artificial Sequence
  source: /note="Description of Artificial Sequence: Synthetic polynucleotide"
accatcaagccttgtcctccatgcaagtgccccgctcctaatctgctcggaggcccttccgtgttcatcttcccacctaagatcaaggacgtgctgatgatctccctgtctcctatcgtgacctgcgtggtggtggacgtgtccgaggatgatcctgacgtgcagatcagttggttcgtgaacaacgtggaagtgcacaccgctcagacccagacacacagagaggactacaacagcaccctgagagtggtgtctgccctgcctatccagcaccaggattggatgtccggcaaagaattcaagtgcaaagtgaacaacaaggacctgcctgctccaatcgagcggaccatctccaagcctggtggcggaggagtggtggaagatctgcggaacgtgacccctcctaaggtgtccctgttcgagccttccaaggccgagatcgccaacaagcagaaagctaccctcgtgtgcctggccagaggcttctttcctgaccacgtggaactgtcttggtgggtcaacggcaaagaggtgcactccggcgtctgtaccgatcctcaggcctacaaagagtccaactactcctacagcctgtcctctcggctgagagtgtctgccaccttctggcacaaccctcggaaccacttcagatgccaggtgcagtttcacggcctgtccgaagaggacaagtggcctgagggatcccctaagcctgtgacacagaacatctctgccgaggcctggggtagagctgatggtggcggaggatctggcggaggtggaagcggcggaggcggatcttctcatctggaacagctgctgatggacctgcaagagctgctgtcccggatggaaaactaccggaacctgaagctgccccggatgctgaccgctaagttcgctctgcctaagcaggccaccgagctgaaggatctgcagtgcctggaagatgagctgggccctctgagacacgtgctggatctgacccagtccaagtcctttcagctcgaggacgccgagaacttcatctccaacatcagagtgaccgtggtcaagctgaagggctccgacaacaccttcgagtgccagttcgacgatgagtccgctacagtggtggacttcctgcggagatggatcgccttctgccagtccatcatctccacctctccacagtgatga

SEQ ID NO: 83 - DNA, 1182 bp, Artificial Sequence
  source: /note="Description of Artificial Sequence: Synthetic polynucleotide"
accatcaagccttgtcctccatgcaagtgccccgctcctaatctgctcggaggcccttccgtgttcatcttcccacctaagatcaaggacgtgctgatgatctccctgtctcctatcgtgacctgcgtggtggtggacgtgtccgaggatgatcctgacgtgcagatcagttggttcgtgaacaacgtggaagtgcacaccgctcagacccagacacacagagaggactacaacagcaccctgagagtggtgtctgccctgcctatccagcaccaggattggatgtccggcaaagaattcaagtgcaaagtgaacaacaaggacctgcctgctccaatcgagcggaccatctccaagcctggtggcggaggaagcgtggtggaagatctgcggaacgtgacccctcctaaggtgtccctgttcgagccttccaaggccgagatcgccaacaagcagaaagctaccctcgtgtgcctggccagaggcttctttcctgaccacgtggaactgtcttggtgggtcaacggcaaagaggtgcactccggcgtctgtaccgatcctcaggcctacaaagagtccaactactcctacagcctgtcctctcggctgagagtgtctgccaccttctggcacaaccctcggaaccacttcagatgccaggtgcagtttcacggcctgtccgaagaggacaagtggcctgagggatcccctaagcctgtgacacagaacatctctgccgaggcctggggtagagctgatggtggcggaggatctggcggaggtggaagcggcggaggcggatcttctcatctggaacagctgctgatggacctgcaagagctgctgtcccggatggaaaactaccggaacctgaagctgccccggatgctgaccgctaagttcgctctgcctaagcaggccaccgagctgaaggatctgcagtgcctggaagatgagctgggccctctgagacacgtgctggatctgacccagtccaagtcctttcagctcgaggacgccgagaacttcatctccaacatcagagtgaccgtggtcaagctgaagggctccgacaacaccttcgagtgccagttcgacgatgagtccgctacagtggtggacttcctgcggagatggatcgccttctgccagtccatcatctccacctctccacagtgatga

SEQ ID NO: 84 - DNA, 1185 bp, Artificial Sequence
  source: /note="Description of Artificial Sequence: Synthetic polynucleotide"
accatcaagccttgtcctccatgcaagtgccccgctcctaatctgctcggaggcccttccgtgttcatcttcccacctaagatcaaggacgtgctgatgatctccctgtctcctatcgtgacctgcgtggtggtggacgtgtccgaggatgatcctgacgtgcagatcagttggttcgtgaacaacgtggaagtgcacaccgctcagacccagacacacagagaggactacaacagcaccctgagagtggtgtctgccctgcctatccagcaccaggattggatgtccggcaaagaattcaagtgcaaagtgaacaacaaggacctgcctgctccaatcgagcggaccatctccaagcctggtggcggaggaagcggtgtggtggaagatctgcggaacgtgacccctcctaaggtgtccctgttcgagccttccaaggccgagatcgccaacaagcagaaagctaccctcgtgtgcctggccagaggcttctttcctgaccacgtggaactgtcttggtgggtcaacggcaaagaggtgcactccggcgtctgtaccgatcctcaggcctacaaagagtccaactactcctacagcctgtcctctcggctgagagtgtctgccaccttctggcacaaccctcggaaccacttcagatgccaggtgcagtttcacggcctgtccgaagaggacaagtggcctgagggatcccctaagcctgtgacacagaacatctctgccgaggcctggggtagagctgatggtggcggaggatctggcggaggtggaagcggcggaggcggatcttctcatctggaacagctgctgatggacctgcaagagctgctgtcccggatggaaaactaccggaacctgaagctgccccggatgctgaccgctaagttcgctctgcctaagcaggccaccgagctgaaggatctgcagtgcctggaagatgagctgggccctctgagacacgtgctggatctgacccagtccaagtcctttcagctcgaggacgccgagaacttcatctccaacatcagagtgaccgtggtcaagctgaagggctccgacaacaccttcgagtgccagttcgacgatgagtccgctacagtggtggacttcctgcggagatggatcgccttctgccagtccatcatctccacctctccacagtgatga

SEQ ID NO: 85 - DNA, 1188 bp, Artificial Sequence
  source: /note="Description of Artificial Sequence: Synthetic polynucleotide"
accatcaagccttgtcctccatgcaagtgccccgctcctaatctgctcggaggcccttccgtgttcatcttcccacctaagatcaaggacgtgctgatgatctccctgtctcctatcgtgacctgcgtggtggtggacgtgtccgaggatgatcctgacgtgcagatcagttggttcgtgaacaacgtggaagtgcacaccgctcagacccagacacacagagaggactacaacagcaccctgagagtggtgtctgccctgcctatccagcaccaggattggatgtccggcaaagaattcaagtgcaaagtgaacaacaaggacctgcctgctccaatcgagcggaccatctccaagcctggtggcggaggaagcggtggcgtggtggaagatctgcggaacgtgacccctcctaaggtgtccctgttcgagccttccaaggccgagatcgccaacaagcagaaagctaccctcgtgtgcctggccagaggcttctttcctgaccacgtggaactgtcttggtgggtcaacggcaaagaggtgcactccggcgtctgtaccgatcctcaggcctacaaagagtccaactactcctacagcctgtcctctcggctgagagtgtctgccaccttctggcacaaccctcggaaccacttcagatgccaggtgcagtttcacggcctgtccgaagaggacaagtggcctgagggatcccctaagcctgtgacacagaacatctctgccgaggcctggggtagagctgatggtggcggaggatctggcggaggtggaagcggcggaggcggatcttctcatctggaacagctgctgatggacctgcaagagctgctgtcccggatggaaaactaccggaacctgaagctgccccggatgctgaccgctaagttcgctctgcctaagcaggccaccgagctgaaggatctgcagtgcctggaagatgagctgggccctctgagacacgtgctggatctgacccagtccaagtcctttcagctcgaggacgccgagaacttcatctccaacatcagagtgaccgtggtcaagctgaagggctccgacaacaccttcgagtgccagttcgacgatgagtccgctacagtggtggacttcctgcggagatggatcgccttctgccagtccatcatctccacctctccacagtgatga

SEQ ID NO: 86 - DNA, 1191 bp, Artificial Sequence
  source: /note="Description of Artificial Sequence: Synthetic polynucleotide"
accatcaagccttgtcctccatgcaagtgccccgctcctaatctgctcggaggcccttccgtgttcatcttcccacctaagatcaaggacgtgctgatgatctccctgtctcctatcgtgacctgcgtggtggtggacgtgtccgaggatgatcctgacgtgcagatcagttggttcgtgaacaacgtggaagtgcacaccgctcagacccagacacacagagaggactacaacagcaccctgagagtggtgtctgccctgcctatccagcaccaggattggatgtccggcaaagaattcaagtgcaaagtgaacaacaaggacctgcctgctccaatcgagcggaccatctccaagcctggtggcggaggaagcggtggcggcgtggtggaagatctgcggaacgtgacccctcctaaggtgtccctgttcgagccttccaaggccgagatcgccaacaagcagaaagctaccctcgtgtgcctggccagaggcttctttcctgaccacgtggaactgtcttggtgggtcaacggcaaagaggtgcactccggcgtctgtaccgatcctcaggcctacaaagagtccaactactcctacagcctgtcctctcggctgagagtgtctgccaccttctggcacaaccctcggaaccacttcagatgccaggtgcagtttcacggcctgtccgaagaggacaagtggcctgagggatcccctaagcctgtgacacagaacatctctgccgaggcctggggtagagctgatggtggcggaggatctggcggaggtggaagcggcggaggcggatcttctcatctggaacagctgctgatggacctgcaagagctgctgtcccggatggaaaactaccggaacctgaagctgccccggatgctgaccgctaagttcgctctgcctaagcaggccaccgagctgaaggatctgcagtgcctggaagatgagctgggccctctgagacacgtgctggatctgacccagtccaagtcctttcagctcgaggacgccgagaacttcatctccaacatcagagtgaccgtggtcaagctgaagggctccgacaacaccttcgagtgccagttcgacgatgagtccgctacagtggtggacttcctgcggagatggatcgccttctgccagtccatcatctccacctctccacagtgatga

SEQ ID NO: 87 - DNA, 1194 bp, Artificial Sequence
  source: /note="Description of Artificial Sequence: Synthetic polynucleotide"
accatcaagccttgtcctccatgcaagtgccccgctcctaatctgctcggaggcccttccgtgttcatcttcccacctaagatcaaggacgtgctgatgatctccctgtctcctatcgtgacctgcgtggtggtggacgtgtccgaggatgatcctgacgtgcagatcagttggttcgtgaacaacgtggaagtgcacaccgctcagacccagacacacagagaggactacaacagcaccctgagagtggtgtctgccctgcctatccagcaccaggattggatgtccggcaaagaattcaagtgcaaagtgaacaacaaggacctgcctgctccaatcgagcggaccatctccaagcctggtggcggaggaagcggtggcggcggagtggtggaagatctgcggaacgtgacccctcctaaggtgtccctgttcgagccttccaaggccgagatcgccaacaagcagaaagctaccctcgtgtgcctggccagaggcttctttcctgaccacgtggaactgtcttggtgggtcaacggcaaagaggtgcactccggcgtctgtaccgatcctcaggcctacaaagagtccaactactcctacagcctgtcctctcggctgagagtgtctgccaccttctggcacaaccctcggaaccacttcagatgccaggtgcagtttcacggcctgtccgaagaggacaagtggcctgagggatcccctaagcctgtgacacagaacatctctgccgaggcctggggtagagctgatggtggcggaggatctggcggaggtggaagcggcggaggcggatcttctcatctggaacagctgctgatggacctgcaagagctgctgtcccggatggaaaactaccggaacctgaagctgccccggatgctgaccgctaagttcgctctgcctaagcaggccaccgagctgaaggatctgcagtgcctggaagatgagctgggccctctgagacacgtgctggatctgacccagtccaagtcctttcagctcgaggacgccgagaacttcatctccaacatcagagtgaccgtggtcaagctgaagggctccgacaacaccttcgagtgccagttcgacgatgagtccgctacagtggtggacttcctgcggagatggatcgccttctgccagtccatcatctccacctctccacagtgatga

SEQ ID NO: 88 - DNA, 1197 bp, Artificial Sequence
  source: /note="Description of Artificial Sequence: Synthetic polynucleotide"
accatcaagccttgtcctccatgcaagtgccccgctcctaatctgctcggaggcccttccgtgttcatcttcccacctaagatcaaggacgtgctgatgatctccctgtctcctatcgtgacctgcgtggtggtggacgtgtccgaggatgatcctgacgtgcagatcagttggttcgtgaacaacgtggaagtgcacaccgctcagacccagacacacagagaggactacaacagcaccctgagagtggtgtctgccctgcctatccagcaccaggattggatgtccggcaaagaattcaagtgcaaagtgaacaacaaggacctgcctgctccaatcgagcggaccatctccaagcctggtggcggaggaagcggtggcggcggatctgtggtggaagatctgcggaacgtgacccctcctaaggtgtccctgttcgagccttccaaggccgagatcgccaacaagcagaaagctaccctcgtgtgcctggccagaggcttctttcctgaccacgtggaactgtcttggtgggtcaacggcaaagaggtgcactccggcgtctgtaccgatcctcaggcctacaaagagtccaactactcctacagcctgtcctctcggctgagagtgtctgccaccttctggcacaaccctcggaaccacttcagatgccaggtgcagtttcacggcctgtccgaagaggacaagtggcctgagggatcccctaagcctgtgacacagaacatctctgccgaggcctggggtagagctgatggtggcggaggatctggcggaggtggaagcggcggaggcggatcttctcatctggaacagctgctgatggacctgcaagagctgctgtcccggatggaaaactaccggaacctgaagctgccccggatgctgaccgctaagttcgctctgcctaagcaggccaccgagctgaaggatctgcagtgcctggaagatgagctgggccctctgagacacgtgctggatctgacccagtccaagtcctttcagctcgaggacgccgagaacttcatctccaacatcagagtgaccgtggtcaagctgaagggctccgacaacaccttcgagtgccagttcgacgatgagtccgctacagtggtggacttcctgcggagatggatcgccttctgccagtccatcatctccacctctccacagtgatga

SEQ ID NO: 89 - DNA, 1344 bp, Artificial Sequence
  source: /note="Description of Artificial Sequence: Synthetic polynucleotide"
caggtgcagctggtggaatctggtggcggagttgtgcagcctggcagatccctgagactgtcttgtgccgcctccggcttcaccttctccagctacaccatgcactgggtccgacaggcccctggcaaaggattggagtgggtcaccttcatctcttacgacggcaacaacaagtactacgccgactccgtgaagggcagattcaccatctctcgggacaactccaagaacaccctgtacctgcagatgaactccctgagagccgaggacaccgccatctactactgtgctagaaccggctggctgggcccctttgattattggggacagggcaccctggtcaccgtgtcctctgcttccaccaagggaccctctgtgttccctctggctccttccagcaagtctacctctggcggaacagctgctctgggctgcctggtcaaggactactttcctgagcctgtgaccgtgtcttggaactctggcgctctgacatccggcgtgcacacctttccagctgtgctgcaatcctccggcctgtactctctgtcctccgtcgtgaccgtgccttctagctctctgggcacccagacctacatctgcaatgtgaaccacaagccttccaacaccaaggtggacaagagagtggaacccaagtcctgcgataagacccacacctgtccaccatgtcctgctccagaactgctcggcggaccttccgtgttcctgtttcctccaaagcctaaggacaccctgatgatctctcggacccctgaagtgacctgcgtggtggtggatgtgtctcacgaggatcccgaagtgaagttcaattggtacgtggacggcgtggaagtgcacaacgccaagaccaagcctagagaggaacagtacaactccacctacagagtggtgtccgtgctgaccgtgctgcaccaggattggctgaacggcaaagagtacaagtgcaaggtgtccaacaaggccctgcctgctcctatcgaaaagaccatctccaaggccaaaggccagcctagggaaccccaggtttacaccctgcctccatgccgggaagagatgaccaagaaccaggtgtccctgtggtgcctggttaagggcttctacccctccgatatcgccgtggaatgggagtctaatggccagcctgagaacaactacaagacaacccctcctgtgctggactccgacggctcattcttcctgtactccaagctgacagtggacaagtccagatggcagcagggcaacgtgttctcctgctccgtgatgcacgaggccctgcacaatcactacacccagaagtccctgtctctgagccccggcaag

SEQ ID NO: 90 - DNA, 1334 bp, Artificial Sequence
  source: /note="Description of Artificial Sequence: Synthetic polynucleotide"
caggtgcagctggtggaatctggtggcggagttgtgcagcctggcagatccctgagactgtcttgtgccgcctccggcttcaccttctcctcttacggaatgcactgggtccgacaggcccctggcaaaggattggagtgggtcgccttcatcagatacgacggctccaacaagtactacgccgactccgtgaagggcagattcaccatctctcgggacaactccaagaacaccctgtacctgcagatgaactccctgagagccgaggacaccgccgtgtactactgcaagacccacggctctcacgacaattggggccagggcacaatggtcaccgtgtcctctgcttccaccaagggaccctctgtgttccctctggctccttccagcaagtctacctctggcggaacagctgctctgggctgcctggtcaaggactactttcctgagcctgtgaccgtgtcttggaactctggcgctctgacatccggcgtgcacacctttccagctgtgctgcaatcctccggcctgtactctctgtcctccgtcgtgaccgtgccttctagctctctgggcacccagacctacatctgcaatgtgaaccacaagccttccaacaccaaggtggacaagagagtggaacccaagtcctgcgataagacccacacctgtccaccatgtcctgctccagaactgctcggcggaccttccgtgttcctgtttcctccaaagcctaaggacaccctgatgatctctcggacccctgaagtgacctgcgtggtggtggatgtgtctcacgaggatcccgaagtgaagttcaattggtacgtggacggcgtggaagtgcacaacgccaagaccaagcctagagaggaacagtacaactccacctacagagtggtgtccgtgctgaccgtgctgcaccaggattggctgaacggcaaagagtacaagtgcaaggtgtccaacaaggccctgcctgctcctatcgaaaagaccatctccaaggccaaagccagcctcgggaacctcaagtctgtaccctgcctcctagccgggaagagatgaccaagaaccaggtgtccctgtcctgcgctgtgaagggcttctacccttccgatatcgccgtggaatgggagagcaatggccagcctgagaacaactacaagaccacacctcctgtgctggactccgacggctcattcttcctggtgtccaagctgacagtggacaagtccagatggcagcagggcaacgtgttctcctgctccgtgatgcacgaggccctgcacaatcactacacccagaagtccctgtctctgagccccggcaag

SEQ ID NO: 91 - protein, 118 aa, Artificial Sequence
  source: /note="Description of Artificial Sequence: Synthetic polypeptide"
QVQLVESGGGVVQPGRSLRLSCAASGFTFSSYTMHWVRQAPGKGLEWVTFISYDGNNKYYADSVKGRFTISRDNSKNTLYLQMNSLRAEDTAIYYCARTGWLGPFDYWGQGTLVTVSS

SEQ ID NO: 92 - protein, 108 aa, Artificial Sequence
  source: /note="Description of Artificial Sequence: Synthetic polypeptide"
EIVLTQSPGTLSLSPGERATLSCRASQSVGSSYLAWYQQKPGQAPRLLIYGAFSRATGIPDRFSGSGSGTDFTLTISRLEPEDFAVYYCQQYGSSPWTFGQGTKVEIK

SEQ ID NO: 93 - protein, 115 aa, Artificial Sequence [sequence omitted]

SEQ ID NO: 94 - protein, 111 aa, Artificial Sequence [sequence omitted]

SEQ ID NO: 95 - protein, 107 aa, Artificial Sequence [sequence omitted]

SEQ ID NO: 96 - protein, 106 aa, Artificial Sequence
  source: /note="Description of Artificial Sequence: Synthetic polypeptide"
GQPKANPTVTLFPPSSEELQANKATLVCLISDFYPGAVTVAWKADGSPVKAGVETTKPSKQSNNKYAASSYLSLTPEQWKSHRSYSCQVTHEGSTVEKTVAPTECS

SEQ ID NO: 97 - protein, 103 aa, Artificial Sequence
  source: /note="Description of Artificial Sequence: Synthetic polypeptide"
ASTKGPSVFPLAPSSKSTSGGTAALGCLVKDYFPEPVTVSWNSGALTSGVHTFPAVLQSSGLYSLSSVVTVPSSSLGTQTYICNVNHKPSNTKVDKRVEPKSC

SEQ ID NO: 98 - protein, 120 aa, Artificial Sequence
  source: /note="Description of Artificial Sequence: Synthetic polypeptide"
DKTHTCPPCPAPELLGGPSVFLFPPKPKDTLMISRTPEVTCVVVDVSHEDPEVKFNWYVDGVEVHNAKTKPREEQYNSTYRVVSVLTVLHQDWLNGKEYKCKVSNKALPAPIEKTISKAK

SEQ ID NO: 99 - protein, 93 aa, Artificial Sequence; identical to SEQ ID NO: 1
  source: /note="Description of Artificial Sequence: Synthetic polypeptide"

SEQ ID NO: 100 - protein, 130 aa, Artificial Sequence; identical to SEQ ID NO: 2
  source: /note="Description of Artificial Sequence: Synthetic polypeptide"

SEQ ID NO: 101 - protein, 1 aa, Artificial Sequence
  source: /note="Description of Artificial Sequence: Synthetic peptide"
G

SEQ ID NO: 102 - protein, 2 aa, Artificial Sequence
  source: /note="Description of Artificial Sequence: Synthetic peptide"
GG

SEQ ID NO: 103 - protein, 3 aa, Artificial Sequence
  source: /note="Description of Artificial Sequence: Synthetic peptide"
GGG

SEQ ID NO: 104 - protein, 4 aa, Artificial Sequence
  source: /note="Description of Artificial Sequence: Synthetic peptide"
GGGG

SEQ ID NO: 105 - protein, 5 aa, Artificial Sequence
  source: /note="Description of Artificial Sequence: Synthetic peptide"
GGGGS

SEQ ID NO: 106 - protein, 6 aa, Artificial Sequence
  source: /note="Description of Artificial Sequence: Synthetic peptide"
GGGGSG

SEQ ID NO: 107 - protein, 7 aa, Artificial Sequence
  source: /note="Description of Artificial Sequence: Synthetic peptide"
GGGGSGG

SEQ ID NO: 108 - protein, 8 aa, Artificial Sequence
  source: /note="Description of Artificial Sequence: Synthetic peptide"
GGGGSGGG

SEQ ID NO: 109 - protein, 9 aa, Artificial Sequence
  source: /note="Description of Artificial Sequence: Synthetic peptide"
GGGGSGGGG

SEQ ID NO: 110 - protein, 10 aa, Artificial Sequence
  source: /note="Description of Artificial Sequence: Synthetic peptide"
GGGGSGGGGS

SEQ ID NO: 111 - protein, 120 aa, Artificial Sequence
  source: /note="Description of Artificial Sequence: Synthetic polypeptide"
TIKPCPPCKCPAPNLLGGPSVFIFPPKIKDVLMISLSPIVTCVVVDVSEDDPDVQISWFVNNVEVHTAQTQTHREDYNSTLRVVSALPIQHQDWMSGKEFKCKVNNKDLPAPIERTISKP

SEQ ID NO: 112 - protein, 114 aa, Artificial Sequence
  source: /note="Description of Artificial Sequence: Synthetic polypeptide"
KPNIQNPEPAVYQLKDPRSQDSTLCLFTDFDSQINVPKTMESGTFITDKCVLDMKAMDSKSNGAIAWSNQTSFTCQDIFKETNATYPSSDVPCDATLTEKSFETDMNLNFQNLS

SEQ ID NO: 113 - protein, 128 aa, Artificial Sequence
  source: /note="Description of Artificial Sequence: Synthetic polypeptide"
VVEDLRNVTPPKVSLFEPSKAEIANKQKATLVCLARGFFPDHVELSWWVNGKEVHSGVCTDPQAYKESNYSYSLSSRLRVSATFWHNPRNHFRCQVQFHGLSEEDKWPEGSPKPVTQNISAEAWGRAD

SEQ ID NO: 114 - protein, 124 aa, Artificial Sequence
  source: /note="Description of Artificial Sequence: Synthetic polypeptide"
SHLEQLLMDLQELLSRMENYRNLKLPRMLTAKFALPKQATELKDLQCLEDELGPLRHVLDLTQSKSFQLEDAENFISNIRVTVVKLKGSDNTFECQFDDESATVVDFLRRWIAFCQSIISTSPQ

SEQ ID NO: 115 - protein, 15 aa, Artificial Sequence
  source: /note="Description of Artificial Sequence: Synthetic peptide"
GGGGSGGGGSGGGGS

SEQ ID NO: 116 - protein, 107 aa, Artificial Sequence
  source: /note="Description of Artificial Sequence: Synthetic polypeptide"
GQPREPQVYTLPPCREEMTKNQVSLWCLVKGFYPSDIAVEWESNGQPENNYKTTPPVLDSDGSFFLYSKLTVDKSRWQQGNVFSCSVMHEALHNHYTQKSLSLSPGK

SEQ ID NO: 117 - protein, 107 aa, Artificial Sequence
  source: /note="Description of Artificial Sequence: Synthetic polypeptide"
GQPREPQVCTLPPSREEMTKNQVSLSCAVKGFYPSDIAVEWESNGQPENNYKTTPPVLDSDGSFFLVSKLTVDKSRWQQGNVFSCSVMHEALHNHYTQKSLSLSPGK

SEQ ID NO: 118 - protein, 434 aa, Artificial Sequence
  source: /note="Description of Artificial Sequence: Synthetic polypeptide"
QVQLVESGGGVVQPGRSLRLSCAASGFTFSSYTMHWVRQAPGKGLEWVTFISYDGNNKYYADSVKGRFTISRDNSKNTLYLQMNSLRAEDTAIYYCARTGWLGPFDYWGQGTLVTVSSASTKGPSVFPLAPSSKSTSGGTAALGCLVKDYFPEPVTVSWNSGALTSGVHTFPAVLQSSGLYSLSSVVTVPSSSLGTQTYICNVNHKPSNTKVDKRVEPKSCDKTHTCPPCPAPELLGGPSVFLFPPKPKDTLMISRTPEVTCVVVDVSHEDPEVKFNWYVDGVEVHNAKTKPREEQYNSTYRVVSVLTVLHQDWLNGKEYKCKVSNKALPAPIEKTISKAKPDIQNPDPAVYQLRDSKSSDKSVCLFTDFDSQTNVSQSKDSDVYITDKCVLDMRSMDFKSNSAVAWSNKSDFACANAFNNSIIPEDTFFPSPE

SEQ ID NO: 119 - protein, 435 aa, Artificial Sequence
  source: /note="Description of Artificial Sequence: Synthetic polypeptide"
QVQLVESGGGVVQPGRSLRLSCAASGFTFSSYTMHWVRQAPGKGLEWVTFISYDGNNKYYADSVKGRFTISRDNSKNTLYLQMNSLRAEDTAIYYCARTGWLGPFDYWGQGTLVTVSSASTKGPSVFPLAPSSKSTSGGTAALGCLVKDYFPEPVTVSWNSGALTSGVHTFPAVLQSSGLYSLSSVVTVPSSSLGTQTYICNVNHKPSNTKVDKRVEPKSCDKTHTCPPCPAPELLGGPSVFLFPPKPKDTLMISRTPEVTCVVVDVSHEDPEVKFNWYVDGVEVHNAKTKPREEQYNSTYRVVSVLTVLHQDWLNGKEYKCKVSNKALPAPIEKTISKAKGPDIQNPDPAVYQLRDSKSSDKSVCLFTDFDSQTNVSQSKDSDVYITDKCVLDMRSMDFKSNSAVAWSNKSDFACANAFNNSIIPEDTFFPSPE

SEQ ID NO: 120 - protein, 436 aa, Artificial Sequence
  source: /note="Description of Artificial Sequence: Synthetic polypeptide"
QVQLVESGGGVVQPGRSLRLSCAASGFTFSSYTMHWVRQAPGKGLEWVTFISYDGNNKYYADSVKGRFTISRDNSKNTLYLQMNSLRAEDTAIYYCARTGWLGPFDYWGQGTLVTVSSASTKGPSVFPLAPSSKSTSGGTAALGCLVKDYFPEPVTVSWNSGALTSGVHTFPAVLQSSGLYSLSSVVTVPSSSLGTQTYICNVNHKPSNTKVDKRVEPKSCDKTHTCPPCPAPELLGGPSVFLFPPKPKDTLMISRTPEVTCVVVDVSHEDPEVKFNWYVDGVEVHNAKTKPREEQYNSTYRVVSVLTVLHQDWLNGKEYKCKVSNKALPAPIEKTISKAKGGPDIQNPDPAVYQLRDSKSSDKSVCLFTDFDSQTNVSQSKDSDVYITDKCVLDMRSMDFKSNSAVAWSNKSDFACANAFNNSIIPEDTFFPSPE

SEQ ID NO: 121 - protein, 437 aa, Artificial Sequence
  source: /note="Description of Artificial Sequence: Synthetic polypeptide"
QVQLVESGGGVVQPGRSLRLSCAASGFTFSSYTMHWVRQAPGKGLEWVTFISYDGNNKYYADSVKGRFTISRDNSKNTLYLQMNSLRAEDTAIYYCARTGWLGPFDYWGQGTLVTVSSASTKGPSVFPLAPSSKSTSGGTAALGCLVKDYFPEPVTVSWNSGALTSGVHTFPAVLQSSGLYSLSSVVTVPSSSLGTQTYICNVNHKPSNTKVDKRVEPKSCDKTHTCPPCPAPELLGGPSVFLFPPKPKDTLMISRTPEVTCVVVDVSHEDPEVKFNWYVDGVEVHNAKTKPREEQYNSTYRVVSVLTVLHQDWLNGKEYKCKVSNKALPAPIEKTISKAKGGGPDIQNPDPAVYQLRDSKSSDKSVCLFTDFDSQTNVSQSKDSDVYITDKCVLDMRSMDFKSNSAVAWSNKSDFACANAFNNSIIPEDTFFPSPE

SEQ ID NO: 122 - protein, 438 aa, Artificial Sequence
  source: /note="Description of Artificial Sequence: Synthetic polypeptide"
QVQLVESGGGVVQPGRSLRLSCAASGFTFSSYTMHWVRQAPGKGLEWVTFISYDGNNKYYADSVKGRFTISRDNSKNTLYLQMNSLRAEDTAIYYCARTGWLGPFDYWGQGTLVTVSSASTKGPSVFPLAPSSKSTSGGTAALGCLVKDYFPEPVTVSWNSGALTSGVHTFPAVLQSSGLYSLSSVVTVPSSSLGTQTYICNVNHKPSNTKVDKRVEPKSCDKTHTCPPCPAPELLGGPSVFLFPPKPKDTLMISRTPEVTCVVVDVSHEDPEVKFNWYVDGVEVHNAKTKPREEQYNSTYRVVSVLTVLHQDWLNGKEYKCKVSNKALPAPIEKTISKAKGGGGPDIQNPDPAVYQLRDSKSSDKSVCLFTDFDSQTNVSQSKDSDVYITDKCVLDMRSMDFKSNSAVAWSNKSDFACANAFNNSIIPEDTFFPSPE

SEQ ID NO: 123 - protein, 439 aa, Artificial Sequence
  source: /note="Description of Artificial Sequence: Synthetic polypeptide"
QVQLVESGGGVVQPGRSLRLSCAASGFTFSSYTMHWVRQAPGKGLEWVTFISYDGNNKYYADSVKGRFTISRDNSKNTLYLQMNSLRAEDTAIYYCARTGWLGPFDYWGQGTLVTVSSASTKGPSVFPLAPSSKSTSGGTAALGCLVKDYFPEPVTVSWNSGALTSGVHTFPAVLQSSGLYSLSSVVTVPSSSLGTQTYICNVNHKPSNTKVDKRVEPKSCDKTHTCPPCPAPELLGGPSVFLFPPKPKDTLMISRTPEVTCVVVDVSHEDPEVKFNWYVDGVEVHNAKTKPREEQYNSTYRVVSVLTVLHQDWLNGKEYKCKVSNKALPAPIEKTISKAKGGGGSPDIQNPDPAVYQLRDSKSSDKSVCLFTDFDSQTNVSQSKDSDVYITDKCVLDMRSMDFKSNSAVAWSNKSDFACANAFNNSIIPEDTFFPSPE

SEQ ID NO: 124 - protein, 440 aa, Artificial Sequence
  source: /note="Description of Artificial Sequence: Synthetic polypeptide"
QVQLVESGGGVVQPGRSLRLSCAASGFTFSSYTMHWVRQAPGKGLEWVTFISYDGNNKYYADSVKGRFTISRDNSKNTLYLQMNSLRAEDTAIYYCARTGWLGPFDYWGQGTLVTVSSASTKGPSVFPLAPSSKSTSGGTAALGCLVKDYFPEPVTVSWNSGALTSGVHTFPAVLQSSGLYSLSSVVTVPSSSLGTQTYICNVNHKPSNTKVDKRVEPKSCDKTHTCPPCPAPELLGGPSVFLFPPKPKDTLMISRTPEVTCVVVDVSHEDPEVKFNWYVDGVEVHNAKTKPREEQYNSTYRVVSVLTVLHQDWLNGKEYKCKVSNKALPAPIEKTISKAKGGGGSGPDIQNPDPAVYQLRDSKSSDKSVCLFTDFDSQTNVSQSKDSDVYITDKCVLDMRSMDFKSNSAVAWSNKSDFACANAFNNSIIPEDTFFPSPE

SEQ ID NO: 125 - protein, 441 aa, Artificial Sequence
  source: /note="Description of Artificial Sequence: Synthetic polypeptide"
QVQLVESGGGVVQPGRSLRLSCAASGFTFSSYTMHWVRQAPGKGLEWVTFISYDGNNKYYADSVKGRFTISRDNSKNTLYLQMNSLRAEDTAIYYCARTGWLGPFDYWGQGTLVTVSSASTKGPSVFPLAPSSKSTSGGTAALGCLVKDYFPEPVTVSWNSGALTSGVHTFPAVLQSSGLYSLSSVVTVPSSSLGTQTYICNVNHKPSNTKVDKRVEPKSCDKTHTCPPCPAPELLGGPSVFLFPPKPKDTLMISRTPEVTCVVVDVSHEDPEVKFNWYVDGVEVHNAKTKPREEQYNSTYRVVSVLTVLHQDWLNGKEYKCKVSNKALPAPIEKTISKAKGGGGSGGPDIQNPDPAVYQLRDSKSSDKSVCLFTDFDSQTNVSQSKDSDVYITDKCVLDMRSMDFKSNSAVAWSNKSDFACANAFNNSIIPEDTFFPSPE

SEQ ID NO: 126 - protein, 442 aa, Artificial Sequence
  source: /note="Description of Artificial Sequence: Synthetic polypeptide"
QVQLVESGGGVVQPGRSLRLSCAASGFTFSSYTMHWVRQAPGKGLEWVTFISYDGNNKYYADSVKGRFTISRDNSKNTLYLQMNSLRAEDTAIYYCARTGWLGPFDYWGQGTLVTVSSASTKGPSVFPLAPSSKSTSGGTAALGCLVKDYFPEPVTVSWNSGALTSGVHTFPAVLQSSGLYSLSSVVTVPSSSLGTQTYICNVNHKPSNTKVDKRVEPKSCDKTHTCPPCPAPELLGGPSVFLFPPKPKDTLMISRTPEVTCVVVDVSHEDPEVKFNWYVDGVEVHNAKTKPREEQYNSTYRVVSVLTVLHQDWLNGKEYKCKVSNKALPAPIEKTISKAKGGGGSGGGPDIQNPDPAVYQLRDSKSSDKSVCLFTDFDSQTNVSQSKDSDVYITDKCVLDMRSMDFKSNSAVAWSNKSDFACANAFNNSIIPEDTFFPSPE

SEQ ID NO: 127 - protein, 443 aa, Artificial Sequence
  source: /note="Description of Artificial Sequence: Synthetic polypeptide"
QVQLVESGGGVVQPGRSLRLSCAASGFTFSSYTMHWVRQAPGKGLEWVTFISYDGNNKYYADSVKGRFTISRDNSKNTLYLQMNSLRAEDTAIYYCARTGWLGPFDYWGQGTLVTVSSASTKGPSVFPLAPSSKSTSGGTAALGCLVKDYFPEPVTVSWNSGALTSGVHTFPAVLQSSGLYSLSSVVTVPSSSLGTQTYICNVNHKPSNTKVDKRVEPKSCDKTHTCPPCPAPELLGGPSVFLFPPKPKDTLMISRTPEVTCVVVDVSHEDPEVKFNWYVDGVEVHNAKTKPREEQYNSTYRVVSVLTVLHQDWLNGKEYKCKVSNKALPAPIEKTISKAKGGGGSGGGGPDIQNPDPAVYQLRDSKSSDKSVCLFTDFDSQTNVSQSKDSDVYITDKCVLDMRSMDFKSNSAVAWSNKSDFACANAFNNSIIPEDTFFPSPE

SEQ ID NO: 128 - protein, 444 aa, Artificial Sequence
  source: /note="Description of Artificial Sequence: Synthetic polypeptide"
QVQLVESGGGVVQPGRSLRLSCAASGFTFSSYTMHWVRQAPGKGLEWVTFISYDGNNKYYADSVKGRFTISRDNSKNTLYLQMNSLRAEDTAIYYCARTGWLGPFDYWGQGTLVTVSSASTKGPSVFPLAPSSKSTSGGTAALGCLVKDYFPEPVTVSWNSGALTSGVHTFPAVLQSSGLYSLSSVVTVPSSSLGTQTYICNVNHKPSNTKVDKRVEPKSCDKTHTCPPCPAPELLGGPSVFLFPPKPKDTLMISRTPEVTCVVVDVSHEDPEVKFNWYVDGVEVHNAKTKPREEQYNSTYRVVSVLTVLHQDWLNGKEYKCKVSNKALPAPIEKTISKAKGGGGSGGGGSPDIQNPDPAVYQLRDSKSSDKSVCLFTDFDSQTNVSQSKDSDVYITDKCVLDMRSMDFKSNSAVAWSNKSDFACANAFNNSIIPEDTFFPSPE

SEQ ID NO: 129 - protein, 108 aa, Artificial Sequence; identical to SEQ ID NO: 92
  source: /note="Description of Artificial Sequence: Synthetic polypeptide"

SEQ ID NO: 130 - protein, 468 aa, Artificial Sequence
  source: /note="Description of Artificial Sequence: Synthetic polypeptide"
QVQLVESGGGVVQPGRSLRLSCAASGFTFSSYGMHWVRQAPGKGLEWVAFIRYDGSNKYYADSVKGRFTISRDNSKNTLYLQMNSLRAEDTAVYYCKTHGSHDNWGQGTMVTVSSASTKGPSVFPLAPSSKSTSGGTAALGCLVKDYFPEPVTVSWNSGALTSGVHTFPAVLQSSGLYSLSSVVTVPSSSLGTQTYICNVNHKPSNTKVDKRVEPKSCDKTHTCPPCPAPELLGGPSVFLFPPKPKDTLMISRTPEVTCVVVDVSHEDPEVKFNWYVDGVEVHNAKTKPREEQYNSTYRVVSVLTVLHQDWLNGKEYKCKVSNKALPAPIEKTISKAKEDLNKVFPPEVALFEPSEAEISHTQKATLVCLATGFYPDHVELSWWVNGKEVHSGVCTDPQPLKEQPALNDSRYALSSRLRVSATFWQDPRNHFRCQVQFYGLSEADEWTQARAKPVTQIVSAEAWGRAD

SEQ ID NO: 131 - protein, 469 aa, Artificial Sequence
  source: /note="Description of Artificial Sequence: Synthetic polypeptide"
QVQLVESGGGVVQPGRSLRLSCAASGFTFSSYGMHWVRQAPGKGLEWVAFIRYDGSNKYYADSVKGRFTISRDNSKNTLYLQMNSLRAEDTAVYYCKTHGSHDNWGQGTMVTVSSASTKGPSVFPLAPSSKSTSGGTAALGCLVKDYFPEPVTVSWNSGALTSGVHTFPAVLQSSGLYSLSSVVTVPSSSLGTQTYICNVNHKPSNTKVDKRVEPKSCDKTHTCPPCPAPELLGGPSVFLFPPKPKDTLMISRTPEVTCVVVDVSHEDPEVKFNWYVDGVEVHNAKTKPREEQYNSTYRVVSVLTVLHQDWLNGKEYKCKVSNKALPAPIEKTISKAKGEDLNKVFPPEVALFEPSEAEISHTQKATLVCLATGFYPDHVELSWWVNGKEVHSGVCTDPQPLKEQPALNDSRYALSSRLRVSATFWQDPRNHFRCQVQFYGLSEADEWTQARAKPVTQIVSAEAWGRAD

SEQ ID NO: 132 - protein, 470 aa, Artificial Sequence
  source: /note="Description of Artificial Sequence: Synthetic polypeptide"
QVQLVESGGGVVQPGRSLRLSCAASGFTFSSYGMHWVRQAPGKGLEWVAFIRYDGSNKYYADSVKGRFTISRDNSKNTLYLQMNSLRAEDTAVYYCKTHGSHDNWGQGTMVTVSSASTKGPSVFPLAPSSKSTSGGTAALGCLVKDYFPEPVTVSWNSGALTSGVHTFPAVLQSSGLYSLSSVVTVPSSSLGTQTYICNVNHKPSNTKVDKRVEPKSCDKTHTCPPCPAPELLGGPSVFLFPPKPKDTLMISRTPEVTCVVVDVSHEDPEVKFNWYVDGVEVHNAKTKPREEQYNSTYRVVSVLTVLHQDWLNGKEYKCKVSNKALPAPIEKTISKAKGGEDLNKVFPPEVALFEPSEAEISHTQKATLVCLATGFYPDHVELSWWVNGKEVHSGVCTDPQPLKEQPALNDSRYALSSRLRVSATFWQDPRNHFRCQVQFYGLSEADEWTQARAKPVTQIVSAEAWGRAD

SEQ ID NO: 133 - protein, 471 aa, Artificial Sequence
  source: /note="Description of Artificial Sequence: Synthetic polypeptide"
QVQLVESGGGVVQPGRSLRLSCAASGFTFSSYGMHWVRQAPGKGLEWVAFIRYDGSNKYYADSVKGRFTISRDNSKNTLYLQMNSLRAEDTAVYYCKTHGSHDNWGQGTMVTVSSASTKGPSVFPLAPSSKSTSGGTAALGCLVKDYFPEPVTVSWNSGALTSGVHTFPAVLQSSGLYSLSSVVTVPSSSLGTQTYICNVNHKPSNTKVDKRVEPKSCDKTHTCPPCPAPELLGGPSVFLFPPKPKDTLMISRTPEVTCVVVDVSHEDPEVKFNWYVDGVEVHNAKTKPREEQYNSTYRVVSVLTVLHQDWLNGKEYKCKVSNKALPAPIEKTISKAKGGGEDLNKVFPPEVALFEPSEAEISHTQKATLVCLATGFYPDHVELSWWVNGKEVHSGVCTDPQPLKEQPALNDSRYALSSRLRVSATFWQDPRNHFRCQVQFYGLSEADEWTQARAKPVTQIVSAEAWGRAD

SEQ ID NO: 134 - protein, 472 aa, Artificial Sequence
  source: /note="Description of Artificial Sequence: Synthetic polypeptide"
QVQLVESGGGVVQPGRSLRLSCAASGFTFSSYGMHWVRQAPGKGLEWVAFIRYDGSNKYYADSVKGRFTISRDNSKNTLYLQMNSLRAEDTAVYYCKTHGSHDNWGQGTMVTVSSASTKGPSVFPLAPSSKSTSGGTAALGCLVKDYFPEPVTVSWNSGALTSGVHTFPAVLQSSGLYSLSSVVTVPSSSLGTQTYICNVNHKPSNTKVDKRVEPKSCDKTHTCPPCPAPELLGGPSVFLFPPKPKDTLMISRTPEVTCVVVDVSHEDPEVKFNWYVDGVEVHNAKTKPREEQYNSTYRVVSVLTVLHQDWLNGKEYKCKVSNKALPAPIEKTISKAKGGGGEDLNKVFPPEVALFEPSEAEISHTQKATLVCLATGFYPDHVELSWWVNGKEVHSGVCTDPQPLKEQPALNDSRYALSSRLRVSATFWQDPRNHFRCQVQFYGLSEADEWTQARAKPVTQIVSAEAWGRAD

SEQ ID NO: 135 - protein, 473 aa, Artificial Sequence
  source: /note="Description of Artificial Sequence: Synthetic polypeptide"
QVQLVESGGGVVQPGRSLRLSCAASGFTFSSYGMHWVRQAPGKGLEWVAFIRYDGSNKYYADSVKGRFTISRDNSKNTLYLQMNSLRAEDTAVYYCKTHGSHDNWGQGTMVTVSSASTKGPSVFPLAPSSKSTSGGTAALGCLVKDYFPEPVTVSWNSGALTSGVHTFPAVLQSSGLYSLSSVVTVPSSSLGTQTYICNVNHKPSNTKVDKRVEPKSCDKTHTCPPCPAPELLGGPSVFLFPPKPKDTLMISRTPEVTCVVVDVSHEDPEVKFNWYVDGVEVHNAKTKPREEQYNSTYRVVSVLTVLHQDWLNGKEYKCKVSNKALPAPIEKTISKAKGGGGSEDLNKVFPPEVALFEPSEAEISHTQKATLVCLATGFYPDHVELSWWVNGKEVHSGVCTDPQPLKEQPALNDSRYALSSRLRVSATFWQDPRNHFRCQVQFYGLSEADEWTQARAKPVTQIVSAEAWGRAD

SEQ ID NO: 136 - protein, 474 aa, Artificial Sequence
  source: /note="Description of Artificial Sequence: Synthetic polypeptide"
QVQLVESGGGVVQPGRSLRLSCAASGFTFSSYGMHWVRQAPGKGLEWVAFIRYDGSNKYYADSVKGRFTISRDNSKNTLYLQMNSLRAEDTAVYYCKTHGSHDNWGQGTMVTVSSASTKGPSVFPLAPSSKSTSGGTAALGCLVKDYFPEPVTVSWNSGALTSGVHTFPAVLQSSGLYSLSSVVTVPSSSLGTQTYICNVNHKPSNTKVDKRVEPKSCDKTHTCPPCPAPELLGGPSVFLFPPKPKDTLMISRTPEVTCVVVDVSHEDPEVKFNWYVDGVEVHNAKTKPREEQYNSTYRVVSVLTVLHQDWLNGKEYKCKVSNKALPAPIEKTISKAKGGGGSGEDLNKVFPPEVALFEPSEAEISHTQKATLVCLATGFYPDHVELSWWVNGKEVHSGVCTDPQPLKEQPALNDSRYALSSRLRVSATFWQDPRNHFRCQVQFYGLSEADEWTQARAKPVTQIVSAEAWGRAD

SEQ ID NO: 137 - protein, 475 aa, Artificial Sequence
  source: /note="Description of Artificial Sequence: Synthetic polypeptide"
QVQLVESGGGVVQPGRSLRLSCAASGFTFSSYGMHWVRQAPGKGLEWVAFIRYDGSNKYYADSVKGRFTISRDNSKNTLYLQMNSLRAEDTAVYYCKTHGSHDNWGQGTMVTVSSASTKGPSVFPLAPSSKSTSGGTAALGCLVKDYFPEPVTVSWNSGALTSGVHTFPAVLQSSGLYSLSSVVTVPSSSLGTQTYICNVNHKPSNTKVDKRVEPKSCDKTHTCPPCPAPELLGGPSVFLFPPKPKDTLMISRTPEVTCVVVDVSHEDPEVKFNWYVDGVEVHNAKTKPREEQYNSTYRVVSVLTVLHQDWLNGKEYKCKVSNKALPAPIEKTISKAKGGGGSGGEDLNKVFPPEVALFEPSEAEISHTQKATLVCLATGFYPDHVELSWWVNGKEVHSGVCTDPQPLKEQPALNDSRYALSSRLRVSATFWQDPRNHFRCQVQFYGLSEADEWTQARAKPVTQIVSAEAWGRAD

SEQ ID NO: 138 - protein, 476 aa, Artificial Sequence
  source: /note="Description of Artificial Sequence: Synthetic polypeptide"
QVQLVESGGGVVQPGRSLRLSCAASGFTFSSYGMHWVRQAPGKGLEWVAFIRYDGSNKYYADSVKGRFTISRDNSKNTLYLQMNSLRAEDTAVYYCKTHGSHDNWGQGTMVTVSSASTKGPSVFPLAPSSKSTSGGTAALGCLVKDYFPEPVTVSWNSGALTSGVHTFPAVLQSSGLYSLSSVVTVPSSSLGTQTYICNVNHKPSNTKVDKRVEPKSCDKTHTCPPCPAPELLGGPSVFLFPPKPKDTLMISRTPEVTCVVVDVSHEDPEVKFNWYVDGVEVHNAKTKPREEQYNSTYRVVSVLTVLHQDWLNGKEYKCKVSNKALPAPIEKTISKAKGGGGSGGGEDLNKVFPPEVALFEPSEAEISHTQKATLVCLATGFYPDHVELSWWVNGKEVHSGVCTDPQPLKEQPALNDSRYALSSRLRVSATFWQDPRNHFRCQVQFYGLSEADEWTQARAKPVTQIVSAEAWGRAD

SEQ ID NO: 139 - protein, 477 aa, Artificial Sequence
  source: /note="Description of Artificial Sequence: Synthetic polypeptide"
QVQLVESGGGVVQPGRSLRLSCAASGFTFSSYGMHWVRQAPGKGLEWVAFIRYDGSNKYYADSVKGRFTISRDNSKNTLYLQMNSLRAEDTAVYYCKTHGSHDNWGQGTMVTVSSASTKGPSVFPLAPSSKSTSGGTAALGCLVKDYFPEPVTVSWNSGALTSGVHTFPAVLQSSGLYSLSSVVTVPSSSLGTQTYICNVNHKPSNTKVDKRVEPKSCDKTHTCPPCPAPELLGGPSVFLFPPKPKDTLMISRTPEVTCVVVDVSHEDPEVKFNWYVDGVEVHNAKTKPREEQYNSTYRVVSVLTVLHQDWLNGKEYKCKVSNKALPAPIEKTISKAKGGGGSGGGGEDLNKVFPPEVALFEPSEAEISHTQKATLVCLATGFYPDHVELSWWVNGKEVHSGVCTDPQPLKEQPALNDSRYALSSRLRVSATFWQDPRNHFRCQVQFYGLSEADEWTQARAKPVTQIVSAEAWGRAD

SEQ ID NO: 140 - protein, 478 aa, Artificial Sequence
  source: /note="Description of Artificial Sequence: Synthetic polypeptide"
QVQLVESGGGVVQPGRSLRLSCAASGFTFSSYGMHWVRQAPGKGLEWVAFIRYDGSNKYYADSVKGRFTISRDNSKNTLYLQMNSLRAEDTAVYYCKTHGSHDNWGQGTMVTVSSASTKGPSVFPLAPSSKSTSGGTAALGCLVKDYFPEPVTVSWNSGALTSGVHTFPAVLQSSGLYSLSSVVTVPSSSLGTQTYICNVNHKPSNTKVDKRVEPKSCDKTHTCPPCPAPELLGGPSVFLFPPKPKDTLMISRTPEVTCVVVDVSHEDPEVKFNWYVDGVEVHNAKTKPREEQYNSTYRVVSVLTVLHQDWLNGKEYKCKVSNKALPAPIEKTISKAKGGGGSGGGGSEDLNKVFPPEVALFEPSEAEISHTQKATLVCLATGFYPDHVELSWWVNGKEVHSGVCTDPQPLKEQPALNDSRYALSSRLRVSATFWQDPRNHFRCQVQFYGLSEADEWTQARAKPVTQIVSAEAWGRAD

SEQ ID NO: 141 - protein, 217 aa, Artificial Sequence
  source: /note="Description of Artificial Sequence: Synthetic polypeptide"
QSVLTQPPSVSGAPGQRVTISCSGSRSNIGSNTVKWYQQLPGTAPKLLIYYNDQRPSGVPDRFSGSKSGTSASLAITGLQAEDEADYYCQSYDRYTHPALLFGTGTKVTVLGQPKANPTVTLFPPSSEELQANKATLVCLISDFYPGAVTVAWKADGSPVKAGVETTKPSKQSNNKYAASSYLSLTPEQWKSHRSYSCQVTHEGSTVEKTVAPTECS

SEQ ID NO: 142 - protein, 234 aa, Artificial Sequence
  source: /note="Description of Artificial Sequence: Synthetic polypeptide"
TIKPCPPCKCPAPNLLGGPSVFIFPPKIKDVLMISLSPIVTCVVVDVSEDDPDVQISWFVNNVEVHTAQTQTHREDYNSTLRVVSALPIQHQDWMSGKEFKCKVNNKDLPAPIERTISKPKPNIQNPEPAVYQLKDPRSQDSTLCLFTDFDSQINVPKTMESGTFITDKCVLDMKAMDSKSNGAIAWSNQTSFTCQDIFKETNATYPSSDVPCDATLTEKSFETDMNLNFQNLS

SEQ ID NO: 143 - protein, 235 aa, Artificial Sequence
  source: /note="Description of Artificial Sequence: Synthetic polypeptide"
TIKPCPPCKCPAPNLLGGPSVFIFPPKIKDVLMISLSPIVTCVVVDVSEDDPDVQISWFVNNVEVHTAQTQTHREDYNSTLRVVSALPIQHQDWMSGKEFKCKVNNKDLPAPIERTISKPGKPNIQNPEPAVYQLKDPRSQDSTLCLFTDFDSQINVPKTMESGTFITDKCVLDMKAMDSKSNGAIAWSNQTSFTCQDIFKETNATYPSSDVPCDATLTEKSFETDMNLNFQNLS

SEQ ID NO: 144 - protein, 236 aa, Artificial Sequence
  source: /note="Description of Artificial Sequence: Synthetic polypeptide"
TIKPCPPCKCPAPNLLGGPSVFIFPPKIKDVLMISLSPIVTCVVVDVSEDDPDVQISWFVNNVEVHTAQTQTHREDYNSTLRVVSALPIQHQDWMSGKEFKCKVNNKDLPAPIERTISKPGGKPNIQNPEPAVYQLKDPRSQDSTLCLFTDFDSQINVPKTMESGTFITDKCVLDMKAMDSKSNGAIAWSNQTSFTCQDIFKETNATYPSSDVPCDATLTEKSFETDMNLNFQNLS

SEQ ID NO: 145 - protein, 237 aa, Artificial Sequence
  source: /note="Description of Artificial Sequence: Synthetic polypeptide"
TIKPCPPCKCPAPNLLGGPSVFIFPPKIKDVLMISLSPIVTCVVVDVSEDDPDVQISWFVNNVEVHTAQTQTHREDYNSTLRVVSALPIQHQDWMSGKEFKCKVNNKDLPAPIERTISKPGGGKPNIQNPEPAVYQLKDPRSQDSTLCLFTDFDSQINVPKTMESGTFITDKCVLDMKAMDSKSNGAIAWSNQTSFTCQDIFKETNATYPSSDVPCDATLTEKSFETDMNLNFQNLS

SEQ ID NO: 146 - protein, 238 aa, Artificial Sequence
  source: /note="Description of Artificial Sequence: Synthetic polypeptide"
TIKPCPPCKCPAPNLLGGPSVFIFPPKIKDVLMISLSPIVTCVVVDVSEDDPDVQISWFVNNVEVHTAQTQTHREDYNSTLRVVSALPIQHQDWMSGKEFKCKVNNKDLPAPIERTISKPGGGGKPNIQNPEPAVYQLKDPRSQDSTLCLFTDFDSQINVPKTMESGTFITDKCVLDMKAMDSKSNGAIAWSNQTSFTCQDIFKETNATYPSSDVPCDATLTEKSFETDMNLNFQNLS

SEQ ID NO: 147 - protein, 239 aa, Artificial Sequence
  source: /note="Description of Artificial Sequence: Synthetic polypeptide"
TIKPCPPCKCPAPNLLGGPSVFIFPPKIKDVLMISLSPIVTCVVVDVSEDDPDVQISWFVNNVEVHTAQTQTHREDYNSTLRVVSALPIQHQDWMSGKEFKCKVNNKDLPAPIERTISKPGGGGSKPNIQNPEPAVYQLKDPRSQDSTLCLFTDFDSQINVPKTMESGTFITDKCVLDMKAMDSKSNGAIAWSNQTSFTCQDIFKETNATYPSSDVPCDATLTEKSFETDMNLNFQNLS

SEQ ID NO: 148 - protein, 240 aa, Artificial Sequence
  source: /note="Description of Artificial Sequence: Synthetic polypeptide"
TIKPCPPCKCPAPNLLGGPSVFIFPPKIKDVLMISLSPIVTCVVVDVSEDDPDVQISWFVNNVEVHTAQTQTHREDYNSTLRVVSALPIQHQDWMSGKEFKCKVNNKDLPAPIERTISKPGGGGSGKPNIQNPEPAVYQLKDPRSQDSTLCLFTDFDSQINVPKTMESGTFITDKCVLDMKAMDSKSNGAIAWSNQTSFTCQDIFKETNATYPSSDVPCDATLTEKSFETDMNLNFQNLS

SEQ ID NO: 149 - protein, 241 aa, Artificial Sequence
  source: /note="Description of Artificial Sequence: Synthetic polypeptide"
TIKPCPPCKCPAPNLLGGPSVFIFPPKIKDVLMISLSPIVTCVVVDVSEDDPDVQISWFVNNVEVHTAQTQTHREDYNSTLRVVSALPIQHQDWMSGKEFKCKVNNKDLPAPIERTISKPGGGGSGGKPNIQNPEPAVYQLKDPRSQDSTLCLFTDFDSQINVPKTMESGTFITDKCVLDMKAMDSKSNGAIAWSNQTSFTCQDIFKETNATYPSSDVPCDATLTEKSFETDMNLNFQNLS

SEQ ID NO: 150 - protein, 242 aa, Artificial Sequence
  source: /note="Description of Artificial Sequence: Synthetic polypeptide"
TIKPCPPCKCPAPNLLGGPSVFIFPPKIKDVLMISLSPIVTCVVVDVSEDDPDVQISWFVNNVEVHTAQTQTHREDYNSTLRVVSALPIQHQDWMSGKEFKCKVNNKDLPAPIERTISKPGGGGSGGGKPNIQNPEPAVYQLKDPRSQDSTLCLFTDFDSQINVPKTMESGTFITDKCVLDMKAMDSKSNGAIAWSNQTSFTCQDIFKETNATYPSSDVPCDATLTEKSFETDMNLNFQNLS

SEQ ID NO: 151 - protein, 243 aa, Artificial Sequence
  source: /note="Description of Artificial Sequence: Synthetic polypeptide"
TIKPCPPCKCPAPNLLGGPSVFIFPPKIKDVLMISLSPIVTCVVVDVSEDDPDVQISWFVNNVEVHTAQTQTHREDYNSTLRVVSALPIQHQDWMSGKEFKCKVNNKDLPAPIERTISKPGGGGSGGGGKPNIQNPEPAVYQLKDPRSQDSTLCLFTDFDSQINVPKTMESGTFITDKCVLDMKAMDSKSNGAIAWSNQTSFTCQDIFKETNATYPSSDVPCDATLTEKSFETDMNLNFQNLS

SEQ ID NO: 152 - protein, 244 aa, Artificial Sequence
  source: /note="Description of Artificial Sequence: Synthetic polypeptide"
TIKPCPPCKCPAPNLLGGPSVFIFPPKIKDVLMISLSPIVTCVVVDVSEDDPDVQISWFVNNVEVHTAQTQTHREDYNSTLRVVSALPIQHQDWMSGKEFKCKVNNKDLPAPIERTISKPGGGGSGGGGSKPNIQNPEPAVYQLKDPRSQDSTLCLFTDFDSQINVPKTMESGTFITDKCVLDMKAMDSKSNGAIAWSNQTSFTCQDIFKETNATYPSSDVPCDATLTEKSFETDMNLNFQNLS

SEQ ID NO: 153 - protein, 387 aa, Artificial Sequence
  source: /note="Description of Artificial Sequence: Synthetic polypeptide"
TIKPCPPCKCPAPNLLGGPSVFIFPPKIKDVLMISLSPIVTCVVVDVSEDDPDVQISWFVNNVEVHTAQTQTHREDYNSTLRVVSALPIQHQDWMSGKEFKCKVNNKDLPAPIERTISKPVVEDLRNVTPPKVSLFEPSKAEIANKQKATLVCLARGFFPDHVELSWWVNGKEVHSGVCTDPQAYKESNYSYSLSSRLRVSATFWHNPRNHFRCQVQFHGLSEEDKWPEGSPKPVTQNISAEAWGRADGGGGSGGGGSGGGGSSHLEQLLMDLQELLSRMENYRNLKLPRMLTAKFALPKQATELKDLQCLEDELGPLRHVLDLTQSKSFQLEDAENFISNIRVTVVKLKGSDNTFECQFDDESATVVDFLRRWIAFCQSIISTSPQ

SEQ ID NO: 154 - protein, 388 aa, Artificial Sequence
  source: /note="Description of Artificial Sequence: Synthetic polypeptide"
TIKPCPPCKCPAPNLLGGPSVFIFPPKIKDVLMISLSPIVTCVVVDVSEDDPDVQISWFVNNVEVHTAQTQTHREDYNSTLRVVSALPIQHQDWMSGKEFKCKVNNKDLPAPIERTISKPGVVEDLRNVTPPKVSLFEPSKAEIANKQKATLVCLARGFFPDHVELSWWVNGKEVHSGVCTDPQAYKESNYSYSLSSRLRVSATFWHNPRNHFRCQVQFHGLSEEDKWPEGSPKPVTQNISAEAWGRADGGGGSGGGGSGGGGSSHLEQLLMDLQELLSRMENYRNLKLPRMLTAKFALPKQATELKDLQCLEDELGPLRHVLDLTQSKSFQLEDAENFISNIRVTVVKLKGSDNTFECQFDDESATVVDFLRRWIAFCQSIISTSPQ

SEQ ID NO: 155 - protein, 389 aa, Artificial Sequence
  source: /note="Description of Artificial Sequence: Synthetic polypeptide"
TIKPCPPCKCPAPNLLGGPSVFIFPPKIKDVLMISLSPIVTCVVVDVSEDDPDVQISWFVNNVEVHTAQTQTHREDYNSTLRVVSALPIQHQDWMSGKEFKCKVNNKDLPAPIERTISKPGGVVEDLRNVTPPKVSLFEPSKAEIANKQKATLVCLARGFFPDHVELSWWVNGKEVHSGVCTDPQAYKESNYSYSLSSRLRVSATFWHNPRNHFRCQVQFHGLSEEDKWPEGSPKPVTQNISAEAWGRADGGGGSGGGGSGGGGSSHLEQLLMDLQELLSRMENYRNLKLPRMLTAKFALPKQATELKDLQCLEDELGPLRHVLDLTQSKSFQLEDAENFISNIRVTVVKLKGSDNTFECQFDDESATVVDFLRRWIAFCQSIISTSPQ

SEQ ID NO: 156 - protein, 390 aa, Artificial Sequence
  source: /note="Description of Artificial Sequence: Synthetic polypeptide"
TIKPCPPCKCPAPNLLGGPSVFIFPPKIKDVLMISLSPIVTCVVVDVSEDDPDVQISWFVNNVEVHTAQTQTHREDYNSTLRVVSALPIQHQDWMSGKEFKCKVNNKDLPAPIERTISKPGGGVVEDLRNVTPPKVSLFEPSKAEIANKQKATLVCLARGFFPDHVELSWWVNGKEVHSGVCTDPQAYKESNYSYSLSSRLRVSATFWHNPRNHFRCQVQFHGLSEEDKWPEGSPKPVTQNISAEAWGRADGGGGSGGGGSGGGGSSHLEQLLMDLQELLSRMENYRNLKLPRMLTAKFALPKQATELKDLQCLEDELGPLRHVLDLTQSKSFQLEDAENFISNIRVTVVKLKGSDNTFECQFDDESATVVDFLRRWIAFCQSIISTSPQ

SEQ ID NO: 157 - protein, 391 aa, Artificial Sequence
  source: /note="Description of Artificial Sequence: Synthetic polypeptide"
TIKPCPPCKCPAPNLLGGPSVFIFPPKIKDVLMISLSPIVTCVVVDVSEDDPDVQISWFVNNVEVHTAQTQTHREDYNSTLRVVSALPIQHQDWMSGKEFKCKVNNKDLPAPIERTISKPGGGGVVEDLRNVTPPKVSLFEPSKAEIANKQKATLVCLARGFFPDHVELSWWVNGKEVHSGVCTDPQAYKESNYSYSLSSRLRVSATFWHNPRNHFRCQVQFHGLSEEDKWPEGSPKPVTQNISAEAWGRADGGGGSGGGGSGGGGSSHLEQLLMDLQELLSRMENYRNLKLPRMLTAKFALPKQATELKDLQCLEDELGPLRHVLDLTQSKSFQLEDAENFISNIRVTVVKLKGSDNTFECQFDDESATVVDFLRRWIAFCQSIISTSPQ

SEQ ID NO: 158 - protein, 142 aa, Homo sapiens
PNIQNPDPAVYQLRDSKSSDKSVCLFTDFDSQTNVSQSKDSDVYITDKTVLDMRSMDFKSNSAVAWSNKSDFACANAFNNSIIPEDTFFPSPESSCDVKLVEKSFETDTNLNFQNLSVIGFRILLLKVAGFNLLMTLRLWSS

SEQ ID NO: 159 - protein, 177 aa, Homo sapiens
EDLNKVFPPEVAVFEPSEAEISHTQKATLVCLATGFFPDHVELSWWVNGKEVHSGVSTDPQPLKEQPALNDSRYCLSSRLRVSATFWQNPRNHFRCQVQFYGLSENDEWTQDRAKPVTQIVSAEAWGRADCGFTSVSYQQGVLSATILYEILLGKATLYAVLVSALVLMAMVKRKDF

SEQ ID NO: 160 - protein, 394 aa, Artificial Sequence
  source: /note="Description of Artificial Sequence: Synthetic polypeptide"
TIKPCPPCKCPAPNLLGGPSVFIFPPKIKDVLMISLSPIVTCVVVDVSEDDPDVQISWFVNNVEVHTAQTQTHREDYNSTLRVVSALPIQHQDWMSGKEFKCKVNNKDLPAPIERTISKPGGGGSGGVVEDLRNVTPPKVSLFEPSKAEIANKQKATLVCLARGFFPDHVELSWWVNGKEVHSGVCTDPQAYKESNYSYSLSSRLRVSATFWHNPRNHFRCQVQFHGLSEEDKWPEGSPKPVTQNISAEAWGRADGGGGSGGGGSGGGGSSHLEQLLMDLQELLSRMENYRNLKLPRMLTAKFALPKQATELKDLQCLEDELGPLRHVLDLTQSKSFQLEDAENFISNIRVTVVKLKGSDNTFECQFDDESATVVDFLRRWIAFCQSIISTSPQ

SEQ ID NO: 161 - protein, 395 aa, Artificial Sequence
  source: /note="Description of Artificial Sequence: Synthetic polypeptide"
TIKPCPPCKCPAPNLLGGPSVFIFPPKIKDVLMISLSPIVTCVVVDVSEDDPDVQISWFVNNVEVHTAQTQTHREDYNSTLRVVSALPIQHQDWMSGKEFKCKVNNKDLPAPIERTISKPGGGGSGGGVVEDLRNVTPPKVSLFEPSKAEIANKQKATLVCLARGFFPDHVELSWWVNGKEVHSGVCTDPQAYKESNYSYSLSSRLRVSATFWHNPRNHFRCQVQFHGLSEEDKWPEGSPKPVTQNISAEAWGRADGGGGSGGGGSGGGGSSHLEQLLMDLQELLSRMENYRNLKLPRMLTAKFALPKQATELKDLQCLEDELGPLRHVLDLTQSKSFQLEDAENFISNIRVTVVKLKGSDNTFECQFDDESATVVDFLRRWIAFCQSIISTSPQ

SEQ ID NO: 162 - protein, 396 aa, Artificial Sequence
  source: /note="Description of Artificial Sequence: Synthetic polypeptide"
TIKPCPPCKCPAPNLLGGPSVFIFPPKIKDVLMISLSPIVTCVVVDVSEDDPDVQISWFVNNVEVHTAQTQTHREDYNSTLRVVSALPIQHQDWMSGKEFKCKVNNKDLPAPIERTISKPGGGGSGGGGVVEDLRNVTPPKVSLFEPSKAEIANKQKATLVCLARGFFPDHVELSWWVNGKEVHSGVCTDPQAYKESNYSYSLSSRLRVSATFWHNPRNHFRCQVQFHGLSEEDKWPEGSPKPVTQNISAEAWGRADGGGGSGGGGSGGGGSSHLEQLLMDLQELLSRMENYRNLKLPRMLTAKFALPKQATELKDLQCLEDELGPLRHVLDLTQSKSFQLEDAENFISNIRVTVVKLKGSDNTFECQFDDESATVVDFLRRWIAFCQSIISTSPQ

SEQ ID NO: 163 - protein, 397 aa, Artificial Sequence
  source: /note="Description of Artificial Sequence: Synthetic polypeptide"
TIKPCPPCKCPAPNLLGGPSVFIFPPKIKDVLMISLSPIVTCVVVDVSEDDPDVQISWFVNNVEVHTAQTQTHREDYNSTLRVVSALPIQHQDWMSGKEFKCKVNNKDLPAPIERTISKPGGGGSGGGGSVVEDLRNVTPPKVSLFEPSKAEIANKQKATLVCLARGFFPDHVELSWWVNGKEVHSGVCTDPQAYKESNYSYSLSSRLRVSATFWHNPRNHFRCQVQFHGLSEEDKWPEGSPKPVTQNISAEAWGRADGGGGSGGGGSGGGGSSHLEQLLMDLQELLSRMENYRNLKLPRMLTAKFALPKQATELKDLQCLEDELGPLRHVLDLTQSKSFQLEDAENFISNIRVTVVKLKGSDNTFECQFDDESATVVDFLRRWIAFCQSIISTSPQ

SEQ ID NO: 164 - protein, 448 aa, Artificial Sequence
  source: /note="Description of Artificial Sequence: Synthetic polypeptide"
QVQLVESGGGVVQPGRSLRLSCAASGFTFSSYTMHWVRQAPGKGLEWVTFISYDGNNKYYADSVKGRFTISRDNSKNTLYLQMNSLRAEDTAIYYCARTGWLGPFDYWGQGTLVTVSSASTKGPSVFPLAPSSKSTSGGTAALGCLVKDYFPEPVTVSWNSGALTSGVHTFPAVLQSSGLYSLSSVVTVPSSSLGTQTYICNVNHKPSNTKVDKRVEPKSCDKTHTCPPCPAPELLGGPSVFLFPPKPKDTLMISRTPEVTCVVVDVSHEDPEVKFNWYVDGVEVHNAKTKPREEQYNSTYRVVSVLTVLHQDWLNGKEYKCKVSNKALPAPIEKTISKAKGQPREPQVYTLPPCREEMTKNQVSLWCLVKGFYPSDIAVEWESNGQPENNYKTTPPVLDSDGSFFLYSKLTVDKSRWQQGNVFSCSVMHEALHNHYTQKSLSLSPGK

SEQ ID NO: 165 - protein, 445 aa, Artificial Sequence
  source: /note="Description of Artificial Sequence: Synthetic polypeptide"
QVQLVESGGGVVQPGRSLRLSCAASGFTFSSYGMHWVRQAPGKGLEWVAFIRYDGSNKYYADSVKGRFTISRDNSKNTLYLQMNSLRAEDTAVYYCKTHGSHDNWGQGTMVTVSSASTKGPSVFPLAPSSKSTSGGTAALGCLVKDYFPEPVTVSWNSGALTSGVHTFPAVLQSSGLYSLSSVVTVPSSSLGTQTYICNVNHKPSNTKVDKRVEPKSCDKTHTCPPCPAPELLGGPSVFLFPPKPKDTLMISRTPEVTCVVVDVSHEDPEVKFNWYVDGVEVHNAKTKPREEQYNSTYRVVSVLTVLHQDWLNGKEYKCKVSNKALPAPIEKTISKAKGQPREPQVCTLPPSREEMTKNQVSLSCAVKGFYPSDIAVEWESNGQPENNYKTTPPVLDSDGSFFLVSKLTVDKSRWQQGNVFSCSVMHEALHNHYTQKSLSLSPGK

SEQ ID NO: 166 - protein, 392 aa, Artificial Sequence
  source: /note="Description of Artificial Sequence: Synthetic polypeptide"
TIKPCPPCKCPAPNLLGGPSVFIFPPKIKDVLMISLSPIVTCVVVDVSEDDPDVQISWFVNNVEVHTAQTQTHREDYNSTLRVVSALPIQHQDWMSGKEFKCKVNNKDLPAPIERTISKPGGGGSVVEDLRNVTPPKVSLFEPSKAEIANKQKATLVCLARGFFPDHVELSWWVNGKEVHSGVCTDPQAYKESNYSYSLSSRLRVSATFWHNPRNHFRCQVQFHGLSEEDKWPEGSPKPVTQNISAEAWGRADGGGGSGGGGSGGGGSSHLEQLLMDLQELLSRMENYRNLKLPRMLTAKFALPKQATELKDLQCLEDELGPLRHVLDLTQSKSFQLEDAENFISNIRVTVVKLKGSDNTFECQFDDESATVVDFLRRWIAFCQSIISTSPQ

SEQ ID NO: 167 - protein, 393 aa, Artificial Sequence
  source: /note="Description of Artificial Sequence: Synthetic polypeptide"
TIKPCPPCKCPAPNLLGGPSVFIFPPKIKDVLMISLSPIVTCVVVDVSEDDPDVQISWFVNNVEVHTAQTQTHREDYNSTLRVVSALPIQHQDWMSGKEFKCKVNNKDLPAPIERTISKPGGGGSGVVEDLRNVTPPKVSLFEPSKAEIANKQKATLVCLARGFFPDHVELSWWVNGKEVHSGVCTDPQAYKESNYSYSLSSRLRVSATFWHNPRNHFRCQVQFHGLSEEDKWPEGSPKPVTQNISAEAWGRADGGGGSGGGGSGGGGSSHLEQLLMDLQELLSRMENYRNLKLPRMLTAKFALPKQATELKDLQCLEDELGPLRHVLDLTQSKSFQLEDAENFISNIRVTVVKLKGSDNTFECQFDDESATVVDFLRRWIAFCQSIISTSPQ

SEQ ID NO: 168 - protein, 90 aa, Artificial Sequence
  source: /note="Description of Artificial Sequence: Synthetic polypeptide"
PNIQNPDPAVYQLRDSKSSDKSVCLFTDFDSQTNVSQSKDSDVYITDKTVLDMRSMDFKSNSAVAWSNKFACANAFNNSIIPEDTFFPSP

SEQ ID NO: 169 - protein, 102 aa, Artificial Sequence
  source: /note="Description of Artificial Sequence: Synthetic polypeptide"
GQPREPQVYTLPPCRDELTKNQVSLWCLVKGFYPSDIAVEWESNGQPENNYKTTPPVLDSDGSFFLYSKLTVDKSRWQQGNVFSCSVMHEALHNHYTQKSLS

SEQ ID NO: 170 - protein, 129 aa, Artificial Sequence
  source: /note="Description of Artificial Sequence: Synthetic polypeptide"
EDLKNVFPPEVAVFEPSEAEISHTQKATLVCLATGFYPDHVELSWWVNGKEVHSGVSTDPQPLKEQPALNDSRYALSSRLRVSATFWQNPRNHFRCQVQFYGLSENDEWTQDRAKPVTQIVSAEAWGRA

SEQ ID NO: 171 - protein, 102 aa, Artificial Sequence
  source: /note="Description of Artificial Sequence: Synthetic polypeptide"
GQPREPQVCTLPPSRDELTKNQVSLSCAVKGFYPSDIAVEWESNGQPENNYKTTPPVLDSDGSFFLVSKLTVDKSRWQQGNVFSCSVMHEALHNHYTQKSLS